European Patent Application EP 4 696 777 A1, published February 18, 2026. Title: Cas13蛋白、CRISPR-Cas系统及其应用. Applicant: 尧唐（上海）生物科技有限公司. Application CN. The sequence listing filed with the application follows.

SEQUENCE LISTING (63 sequences)

SEQ ID NO: 1 - protein, 519 aa, unidentified
MRIVRPYGQSVTRAIGSGRAEQRRLLRLREALHAVEGGALERDLIAFAGTHDALVIAQWISTIDKIATKPRGSKRPTAMQRDLRQELGEAAWAHLVQARLLPGLDGDGAAWLEKLWRFKVHPYPDGLAKPERTRDGRPKEPPSPRGRWYARFAGDVEPAEIDAAAVVQRIHEHLHVAAYRMALGRPVKRLGQIEARARSIAGNVPRPDAGTGVALTWTTAGDAYVARVGNIAEQIREAALAREAGEDGAGTRRVGPDVAARVLHAAWADLFDGSRPSFEEARQRQPELVALHEAIRDRYSRTLKRHGKDRREHRDQRRQVSDLLPRSMPALFALLDATARNRDLAGLVRLGKVIHYEAAARAGGSEPGDAPAHVLTHWPTDVRESHSWTSDGQAAIKRNEAFVRIWRHGLALARQTLTDWADPKGTLDADILLAAGIDQATSRKRFDPAHHERKLNVLLGSRASLFIDGRSDDFRKGTLRLALEGIAQLRHNAFHFNGLAGFTQALRLTKPKPTSCVPL

SEQ ID NO: 2 - protein, 726 aa, unidentified
MTQLWSADLEGRTVRLLQTMGAAHFAGFLDEAQNQMLLDAFFGAMDGANEAALPSVPLPRFRRLLTRAANIAGKGGTVLRLPEPVNRDMLERWPARLCQYVALKLLYDHPFRDWLGRLDTAALNGLIDRAVNRTEAEARKINARKDDADRRALITARARQIGRLGAGESIQGFLFRLSAETASEMRVQSGYESDSELAREQAGYIEDLRCDVLALAFDHYIGEAGFRFLTELPAEAELPAEPLCNLARLRRAEVDASVEDWQAVLYFLLHLVPVDDIGRLLHQIRKWDLLAGGNDGAAEADSSIATRERVRQIMRTLGLYLDMHDAKFEGGAALAVLATYKELFETETSFDRLFPAPISPLDDGRVPRRGLREIMRFGHLPTLLAIFHRYTVRDAEVKALLAAETATDGPSAVADAQSERERLHDDWSGDRKRFTGDACRRYVEALVVVMRHRHSAAHVMLGNHVRLHRLMMAVLGRLVDFSGLWERDLYFSILALMHREGLTPREVFKDRGLEMLSGGQVVAARRNLVAPGIEAELARHFGRSDDERIKVRNDLAHFNMINAAKSDGQPPDLTACVNAARRLVDHDRKLKNAVSQSVIELLKREGIDLTWEMDASAGGHRLTNARIAVRQATHLGGMKLPEAANARGSGRPRFHLIKESLHGDRLGDMVAELFAGVRVPAGIDVSGIPMERIAWNEVNQPRKTGPKRPGAPTGRTHPGRRWRGNQ

SEQ ID NO: 3 - protein, 1125 aa, unidentified
MNEEIKKRSFQEHPQYFGAFLNMARLNIFSISNHLALIFNQADLKDEETILTSFLANKNAKKLNWNRVMGALQKFMPIVKLFNNETLPKSEKEKLKAENKYQPKNDYEKMCGFLFKLFKEISDFRNDYTHYYSIENKTIRKKTVDNEIKDFLIENFDRAVEYTKTRFANVFSDEDFESFHKIKLFEDNSEITSLGLVFLTSLFLEREYAFLFIGKVTGLKGTQYKSFLAVRETFMAFCVKLPHEKFVSEDKKQALSLMIINELNKCPQTLFDVITEEQKVEFRPLLDIVAKANILENSVPEDENDYDTYIQNITKKVRNENRFAYFALKYIDEANVFNKFRFQINLGKILLSEYTKKIANEELDRQIIDKAFAFGKLNSFTDQENEILAKINRANGSIEFEQFAPHYNFNEKSFKIGISSKESNSIFINKENKAKGVLKQPVPEAFLSLNSIDKIVLLDYLKKGESEKLINDFIKINNSTILNWEFIENIKSKFADLPVFKKFSKNKKQNSAYDDEKLCELIERKNNLNKVLAQYQLNYKQIPSRIVEYWLNIQDTSNIRKFSDRIKLMKNEGKERLKNLQKNKSPKVGEMATFLAKDIVDMIISKDVKDKFTSFYYDKLQECLALYNVPEKKQMFLDICKMPEFNLFDTKKGHPFLAKIRPENIKYTTNFYKVYLEEKTLKMVETFNFKKNKTTKKDQSWMFTTFYTLEYSEKAGKKMTVVKIPASTINLPFTIKQWSKERPDLKKWFENIHGKIDNAPKPIKKPIDLPTNLFDAEIKNDLQHSLIQNQIPYNETDTNNQLFKLWWTKVKNNGFMKFYNAKREYCIYDEYVNFEIKPQGKFADYYKSALKTAFEKLDKQRETERIANKALPKVQIKQVEKVFKQTIGNTEKEIRILQEQDALMLLMFEKLLNNPNPNILENISMENILNESIDVKIEINGKLSFENEGEIIKKNENKPQISRIIVEKRKRKEFSVLQKYLHDKRLPELFEYFDKQEIPVSELKLELDTYNQVKNQVFDLVFRFEKTLIEKDYEGIKSFIETKTGEEPKNHIQHKPYLFWLKSKNFIDENEFRFLNMVRNTFSHNQFPQKKTMDLFITQWENNKFANAIFEFYKGKVENILNILM

SEQ ID NO: 4 - protein, 1403 aa, unidentified
MNTTDKRTKPNYKDFINDKDYFSAYLNMARHNAYITVAHISHLLGGKPSGDDAKIMEMKAMQVLQGTDNIEKQKCIRQLNKHFKFLPAVVYYEKLWEKKKAENRFDILDSELDTEESFDLQDSKQQLSEGNIYYSVLSKLFEPLNDLRNFYTHYYHPVVVVPNYVFGFMNKIFDASVRICKQRFGYNEKDIKHLRRYDGSETDSTGKRMPKENPRFFFKINEPNGTITEKGLAFYICLFLEKKYASNFLKKLTGFKDARTADKQSTFEVYTALRMHLPKQRIRSEETKLGIALDMLNELQKCPDELYELLSDENQDKFRVEVTMRSDADDYEENGLFKRFDNRFPYFALKYFDFRAGFPIRFHVDMGKYYFKFYEKKLVNGSTEIRKLDKDLRAFGRIAELDEYRKNEWAELIKANPVNTENFDFDTATSDKYQPYIQDTYPHYHIEDNQIGLKFTEVDIVPEINAEKTRNQKPDAYLSTYELAGMFFYDWLNKNKEQSASAVLLKEYYDKVRKLFEDIGNDTIKPINFQFTANANDEIWQNELKQAKIQANEIISKSYNLDIHNLPEIIQRHLIGLSIIKDDAFKIYAVDRINKMLGETESRLKKLDKGIRIANDKKIKFGSKRFKEIKSGVLADFLAKDLIRFQPTEQNGKDKITGLNFQILQAHLATFNENKHLLPSIFKECKLTDSVIQHPFLFKLNPSKHLDHISFCKAYLVERKFYLQKCLKEAKFNSYYFLQQKRKNLNERKQSNFIKNVTKKYLNEHPINFPRGLFCEAIRSMIKKDSFSHFKNLNPKASETSIRNFLELTQNRTNTVFLIQKYFELLRGDESQEFYQYERSYKFINQLYDRRDRNQMTKELPQLFYPVKDVVENGRLITEGLVSIVDKLKKDIKKLPPIPQTIKSLRFGEKPPMYKESMMAQYNQFKKNEAKLRLYKVQDMLILLIAEHLLELENINIPSGLFLLKNILPPDLVNPVDDKKNILNYPVRYPINLQFKNLPVATIYQNGLKIKNVGDFVRFTRDRRIEGLLDWYRIDYFKPKDANGNIVVDKKGKHLLYKGTDKFVYEINRLFIENEFSVYEKLRIVVLQNVLTFEKVMHDLYKPELIAELAAENVRLKTKFDAEEAEKKANAESKGEIYIVKQYSEIKYFDFKVVTNVFYNKYHQFTHERDAVVHLRNKFAHNEFPEKSVLTQLDVFQKIVDDYPNSIEYANEKQARIDNTPDMPDDEKRIERLRIEQLRSITDKIAQQSRILFEKYIAEIKREEISAEAETLFNTLIKNLNSNSLAKISTAIQTTYPAENTPLTMYSSAFAEDSKAVISFRYYSDSHPETETTDVSQNINSIISNANSLGLYYFNESLRFFLNNAQPEFEIETINSVKYPDLGDLFNTQIIGKYSQKIGKNNE

SEQ ID NO: 5 - protein, 1067 aa, unidentified
MENKTESLSKTIQGNPAYFGVYLNMARHNILLVDNHLDKKFNQKNSITDDEKISDSFLTRTKSDNPNHLYSELIRYIPCCSIYDPEFMVTNKEKKEDMAIIASIEKGKDFTTMPVHLKAVFKDINQLRNSYTHYGHTDNNWERKAKISTETKEFLERVYSKAINYSQKRFKNVIPDEEFTKLTNLPIFLQNEPSTLTQDGLIFLTSLFLEREFMFYFINQCHGLKNATSLSFKSKRELFGVFCLRLPHEKIISDDPKNALFLDVLNEINKVPKEIFNHLLPEQQKEFRPDFSDERNEKIAENSIREDEEDLDTYIQELQNQYRRGQRFYYLATRLIDELKMLPDFRFQIRIGKYLKKSGQKKFGNDMVKREIIDDIFGFGRLAEFMDEQKITTAINIDKVEDQRFESFAPSYDLKANKVQIKLFAGSNTALDVEKINKDGKTVGYTYSNKVFSISIHELVKILILEYFEPKAANQIIKDFINKNRFISDIKEIEKLKAELASMDNKYRIYEDKNTSPERLSQYKEMMADRTSLLDAALIKFGLDSQSIPRALVDYLISVKPSNRSFAMVRKIKEVKNEARQKVSDYDEYIRPKIGEMATEIAKDIIDMIISKEKKERCTSFYYDKMQEALALYASDEKRELFAQIVKDLNLLDEKQGHPFLKYVSFKSFTKTGEFYRAYFYAKAGKKGERGQDGSWMYRTFYTFDRKTKKTTIQVPNEGLPYIFTRLQKPHGIADLQSWVNNFNKTAIDLPTNIFDKKIEEALKSELLKIGKVSDGNEKWSELFKKWYQSQGLLQPFYNLERTYHVYDYDFKAGSDYDDAYKNKIEQLALKISQDKKKEAKGKFDMQYTKQKIKQLLHKEITHNERGIREIVEQDIVLAINLEVPYQIRDLHKIKEHLNETILLSEKVEDKKIEATRKRKDYGLLNKIRHDKRLKSLFTYIVAETVEYETVKSLLKEYNDVRIKIFDHVFALENLILSKYKNEVVQEQKSTYGPNDTNIKHDPYLNVLLTKGIITDTEKEILKTIRDKFSHNEVPVLDEVDKDCIFESMYRIHATIINKITDSLTTH

SEQ ID NO: 6 - protein, 968 aa, unidentified
MFLYKNEANELISKIKGFKRSDDNTFRSKRNLFSFYSKKFSSQDIDSEEGNLIKFRDIVQYLNLYPKHWNSELEFDAKIPQMTKPLKDKIVEMEIERCFPKKDEKDELFYPKYDRLFNDSYEKFKIYAKYQIFGKKFLGKVIENEYIKQDFSDFELDIFSFEINKTKKYKDSFRKEKSFEKRKKDLEYKSFHKKSEEDFLKNYQKNLKDIQRIIEEEKENLNLDTQKLQKRIAQNMLHVQYGRNQDRFMDFAIRFLAEKKYFGNEAEFKIYQFHTTDEQNNCLATQGKVLTKKEFDNLKYHQGKLVVYKSFEEHLKKYPDWDTPFVIENNSFHVKINFCCASKIICIQRNALIYLLEHALYGNNAQTIENAGKELLIKYFVENETAFDKKYNILKTNTEISKDEKTELKKFFPKRLLHNYYKDETSVKKTKTSSLQKILDDANEAETRYQKLLVKVKREETEYKAKYPEDDTVALVANFEKRNKGKQFKLRFMRKAWQLMYFKDAYLKQIQADNKHHKSYNISRDEFNDFSKWLYAFEEIPVYKEYLSDMFAQKTFFVNKEFKDLFDRSTTFENLYSKTKERYTNWLKTNDTALQKTFELKNYETLLSRTTLFININRFIDFLVREGKLTKNSENMFEYKSLENWGYLIEKYYFKEKLEKTEYKTCGKLFNKLRTVKLEDCLLYEMAIDYLQTDKTIADHAKKHIRVLQTKDVIIEVPDINTNNGGLFKLEIPFNKLMAFEELFKQKEEEENEPKNRKTSFLSNIQIYLKKLKEMSEKTKDKREIEKGISDTVTYFNANKGLKFEHLNKIYSHLISTSAKFTKVELELEKYFIVKNKVEIPNHENRITFDDIDAKKEKVLSKYFDKTIRKKAFHFGVPIIENKPFTYKEKLDEIEIKFIQNEVKPLNKKSFDEYEPEMKSVLIALLETLHDAFYEKNYYENGKKREKDGKKKVADAKNKYFNEVIIKK

SEQ ID NO: 7 - protein, 543 aa, unidentified
MADFVARDMIRLQKNIGKDGGKPNSTEFQILQAKLAFFGKNKDTLHDTFKLFKLIDSENQHPFLNKIDINSTNGILDFYKEYLSQRKKYLEQCISEKKYDEYHFLKLGDKQKQSGQKHIEELATKLKNEVVMNLPRGLFLKPILEALKSSEKTNKLALELENTGRVNTAYIIDQYFTKIMNDKSQELYGYSKSYEFLNKIFDNRKEDKMRNTLPSKYFTTEELTKMTINNEIENKLHESITKQIKKKRINNEIEIERIKEVYKKGYKYFTNNEKQIRLVKTTDKILFMMADEVFRKEFVTDNGLIKSRKNNSSQYQTSVSIDIGYKLAEIRPDSDKGILSLRTKVSLIMPYTYETKKDKIVGLDNAKSIRSENKIKTIVNETIKIKNYGNFRGFLKDRRISSLMPYITDNEVQFEAVKKELEEFGKARIEIFKKIYEFEKIVIKEKELNLNAIPYINHGDILKSLIDEKDERFIIIKQLRDAFSHSNYPDYLLFENDINGEGFNELKNYTSKRKDILNNSIAYQFKNLTIKYYDELIKLATGK

SEQ ID NO: 8 - protein, 845 aa, unidentified
MNEEWKKRFLPKLEEQQKENLQKNSSPAEEEIENYDKFMELLTKQVRHADRFSIFAMRFIDEMQLFDTWRFHINLGKILLASYQKHLNGEDVDRLIVEDVKAFGRLNDYPYESKIINKINRTDDPMVKFEQFVPHYHAENNKIGLCRNRKTLGPVMIENQDAQSKNKRNIKQPHPEVFLSLHELPKIILLEYLKKGETERLINEFVALNNSSLMNREFIDEIKTKVPQDWNGFQKKTSSEKSSGYREEALKYLQGRKKILNDVLAAYNLNDRQIPTKILNYWLNIQDVPLDRVLSERIKKMRKDCKQRLKALRKYRREGKGRIPKVGEMASFLAKDIVDMVIGEEKKKKITSFYYDKMQECLALYADPEKKALFIDIVNNELHLNETDGHPFLKNVPRSEVSYTTDIYERYLEEKGYKEIEVTNEKTGKRTKRDVSWMEKTFYKKERDPKTGKLKTNVGIFSDGNAIPLTIRRSSEKISESLDDWLAHVKNGFKPIDGSRPIDLPTNLFDETINALLKNDLKKHNVLSSEDAKWNELFKLWWSEVRKDSTQDYYTAPREYMIYDEKVCFSNTGKGKYSEYYGSAVEAAYSKKNAEQEEKRKKNPRLPKIERCQIEKVFSKTIGKTEKEIRIVEEKDRSLLLMIEQLLSDQGAKTENLKLKEYVRLLDQEVTIRIPFPVPQQKEGEACPEKDIVTKRKRKDYGALQRFISDRRLPGLYEYFPGDEIPMDDLEVELDAYNKAKQNVLDRAFQLEKNIIDRDMVRVSELFGKISNIQHKPYVDWLKEKSLIDEEIDSFLNAVRNKFSHNEYPPKGIMENVIKKWDEKAYASQIEEAYSQEINKILMQL

SEQ ID NO: 9 - protein, 849 aa, unidentified
MCRLKNGRLRAAIFAKIVIFWYQNFRMRLHVNKSKMKQGSVFNAATDKIPFAIFFNRAQERLNGWYGSLDSINADITVSKQDFTSWFKQFKSEEGNMMPEKRQLVKDKVIARLKDVFRFADYLFRWNMSNSILKLIDKLNDLRNFFSHGYHRPVEWSEYEIDTLNKLYFSLSEYRPKLNRQNLENCLLFDENKTLSYQGAIFFVSLFLTKEDVNQLFDLIYFCFRAEKNLPADSLPHRFLNFNPRREIYTFWNRRGDASLMPDNRQLKKFYDIVSFLRKCPEESLTPETEKLAEKYGVRESDKFIRHAMDYLSDFKALPNLEFFPYKNKKEIFRGNTLFLLRDDKHGCLKGMMGEEVLTRVLVRLFSGIPGTSIETEIREFIRTYYENSLLTIDSFTHPVPKSVDRKRKIAEGDNLLFEVLDERILRRLEFISYRLKDLKRESTSFSESQKADFIVRRWNRWIMYNFKKADGVDKSIKNIQFIKLRAQLTNFRKFKREIINELAASGYDKVYPIKELLEESDLETLYKKTIEYDGKFCDKFLANENERRKKAEAICKYVGLRPIKIGVSESNMSKMPVPIAPKAISCDRLKFEKTLVDLIDEYYPIRTGLNKTHKDNKPAISKERRVNKKYWKLKQRDSLLALIASEYLRNGIKKTAEIGRISLYRFDEDIVELKLKLDYTLQFEDKTADTIKAKKLSFTFDEFAKSRNRMILGGLKDIAFSNKFPDNEIDYSHIEPELETYLYSQIEFMRKILELEERLLKQKPELKVLSKKYVPFGDIEKNLDNLSRHFDKFKAAYPTDMTHIDNLRRIFRNSALHMSVPKIDDKVLVGYFQQGIDFINYYIEQQFG

SEQ ID NO: 10 - DNA, 570 bp, unidentified
  source 1..570: mol_type = other DNA
ccgctctgttcgctctgctggacgctacagccaggaacagggaccttgccggcttagtgaggctgggcaaggtgatccactacgaggctgctgctagggctggaggctctgaacctggagatgctcctgctcacgtgctgacccactggcccaccgatgttagggagagccacagctggacctctgacggacaggctgccatcaagaggaacgaggccttcgtgaggatctggaggcacggcttagccctggctaggcagaccttgaccgattgggctgaccctaagggcaccctggacgccgatatccttttagccgctggcatcgaccaggccacctctaggaagagattcgaccccgctcaccacgagaggaagctgaacgtgctgcttggaagcagggccagcctgttcatcgacggcaggagcgatgacttcaggaagggcaccctgaggctggccttagagggcatcgcccaattgaggcacaacgccttccacttcaacggcctggccggcttcacccaggctttgaggctgaccaaacccaagcctaccagctgcgtgcccc

SEQ ID NO: 11 - DNA, 2178 bp, unidentified
  source 1..2178: mol_type = other DNA
atgacccagctgtggagcgccgacctggagggcaggaccgtgaggttattacagaccatgggcgctgcccacttcgccggcttcctggatgaggctcaaaaccagatgctgctggacgccttcttcggcgccatggacggcgccaatgaagctgctttgccctctgtgcccttacccaggttcaggaggctgctgaccagggctgctaacatcgccggcaaaggcggaacagtgctgaggcttcccgagcctgtgaatagggacatgctggagaggtggcccgctaggctgtgccagtacgttgctctgaagctgctgtacgaccaccccttcagggactggctgggcaggcttgatacagccgccttgaacggactgatcgacagggccgtgaacaggaccgaggctgaagccaggaagatcaacgccaggaaggacgacgccgacaggagggccctgattacagctcgagctaggcagatcggaaggctgggcgctggagagagcatccaaggcttcctgttcaggctgagcgctgagaccgccagcgagatgagggtgcagtctggctatgagagcgacagcgagctggccagggagcaagctggctacatcgaggaccttaggtgcgacgtgctggccctggctttcgaccactacatcggagaagccggattcaggttcctgaccgagctgcccgccgaagctgagttacctgccgagcctttgtgcaacctggctaggctgaggagggccgaggttgatgccagcgttgaagactggcaggccgttctgtacttcctgctgcacctggtgcccgtggacgacatcggaaggctgcttcaccagatcaggaagtgggacctgctggccggcggaaatgatggcgctgctgaagctgacagctctatcgccaccagggagagggtgaggcagatcatgaggaccctgggcctgtacttggacatgcacgacgccaagttcgagggaggagctgctctggccgttctggccacatacaaggagctgttcgagacagagaccagcttcgacagactgttccccgcccctatcagccccttggatgatggaagggttcctaggaggggcttgagggagatcatgaggttcggccacctgcccaccctgcttgctatcttccacaggtacaccgtgagggacgccgaggtgaaggccttactggctgctgagaccgctacagacggacccagcgctgttgctgacgctcagagcgaaagagagaggctgcacgacgactggagcggcgataggaagaggttcaccggcgatgcttgcaggaggtacgtggaggccctggtggttgtgatgaggcacagacacagcgctgcccatgtgatgctgggcaaccacgtgaggctgcacaggctgatgatggccgttctgggaaggctggtggacttcagcggcctgtgggaaagggatctgtacttcagcatcctggccctgatgcacagggagggcctgacccctagggaagtgttcaaggacagaggcctggagatgctgagcggcggccaagttgttgctgctaggaggaacctggtggctcctggcatcgaggccgagttagctaggcacttcggcagaagcgacgacgagaggatcaaggtgaggaacgacctggcccacttcaacatgatcaacgccgccaagagcgatggccagcctcccgacttaacagcctgcgtgaatgccgctaggaggctggtggaccacgacaggaagctgaagaacgccgtgagccagagcgtgatcgagctgctgaagagggagggcatcgacttgacctgggagatggacgcctctgctggaggacacaggctgaccaacgctaggatcgccgttaggcaggccacccaccttggaggaatgaagctgcccgaagctgccaacgctaggggctctggaaggcctaggttccacttgatcaaggagagcctgcacggcgacaggctgggcgatatggtggccgagttgtttgctggagtgagggtgcccgctggcatcgacgtgtctggcatccctatggaaaggatcgcctggaacgaggtgaaccagcccaggaagaccggccctaaaaggcctggcgctcctacaggaaggacacatcctggaaggaggtggaggggaaaccag

SEQ ID NO: 12 - DNA, 3373 bp, unidentified
  source 1..3373: mol_type = other DNA
atgaacgaggagatcaagaagaggagcttccaggagcatccccagtacttcggcgccttcctgaacatggccaggctgaacatcttcagcatctccaaccacctggccctgatcttcaaccaggccgacctgaaggacgaggagaccatcctgaccagcttcctggccaacaagaacgccaagaagctgaactggaacagggtgatgggcgccctgcagaagttcatgcccatcgtgaagctgttcaacaacgagaccctgcccaagagcgaaaaggagaagctgaaggccgagaacaagtaccagcccaagaacgactacgagaagatgtgcggcttcctgttcaagctgttcaaggagatcagcgacttcaggaacgactacacccactactacagcatcgagaacaagaccatcaggaagaagaccgtggacaacgagatcaaggacttcctgatcgagaacttcgacagggccgtggagtacaccaagaccaggttcgccaacgtgttcagcgacgaggacttcgagagcttccacaagatcaagctgttcgaggacaacagcgagatcacctccctgggcctggtgttcctgaccagcctgttcctggagagggaatacgccttcctgttcatcggcaaggtgaccggcctgaagggcacccagtacaagagcttcctggctgtgagggagaccttcatggccttctgcgtgaagctgccccacgagaagttcgtgagcgaggacaagaagcaggccctgagcctgatgatcatcaacgagctgaacaagtgccctcagaccctgttcgacgtgatcaccgaggagcagaaggtggagttcaggcccctgctggacatcgtcgccaaggccaacatcctggagaacagcgtgcccgaggacgagaacgactacgacacctacatccagaacatcaccaagaaggtgaggaacgagaacaggttcgcctacttcgccctgaagtacatcgacgaggccaacgtgttcaacaagttcaggttccagatcaacctgggcaagatcctgctgagcgagtacaccaagaagatcgccaacgaggagctggacaggcagatcatcgacaaggccttcgctttcggcaagctgaacagcttcaccgaccaggagaacgagatcctggccaagatcaacagggccaacggcagcatcgagttcgagcagttcgcccctcactacaacttcaacgagaagagcttcaagatcggcatcagcagcaaggagagcaacagcatcttcatcaacaaggagaacaaggccaaaggcgtgctgaagcagcccgttcccgaggctttcctgagcctgaacagcatcgacaagatcgtgctgctggactacctgaagaagggcgagtccgagaagctgatcaacgacttcatcaagatcaacaacagcaccatcctgaactgggagttcatcgagaacatcaagagcaagttcgccgacctgcccgtgttcaagaagttctctaagaacaagaagcagaacagcgcctacgacgacgagaagctgtgcgagctgatcgagaggaagaacaacctgaacaaggtgctggcccagtaccagctgaactacaagcagatccccagcaggatcgtggagtactggctgaacatccaggacaccagcaacatcaggaagttcagcgacaggatcaagctgatgaagaacgagggcaaggagagactgaagaacctgcagaagaacaagagccccaaggtgggcgagatggccaccttcctggccaaggacatcgttgacatgatcatcagcaaggacgtgaaggacaagttcaccagcttctactacgacaagctgcaggagtgcctggccctgtacaacgtgcccgagaagaagcagatgttcctggacatctgcaagatgcccgagttcaacctgttcgacaccaagaagggccaccccttcctggccaagatcaggcccgagaacatcaagtacaccaccaacttctacaaggtgtacctggaggagaagaccctgaagatggtggagacctttaacttcaagaagaacaagaccaccaagaaggaccagagctggatgttcaccaccttctacaccctggagtacagcgagaaggccggcaagaagatgaccgtggtgaagatccccgccagcaccatcaacctgcccttcaccatcaagcagtggagcaaggagaggcccgacctgaagaagtggttcgagaacatccacggcaagatcgacaacgcccctaagcccatcaagaagcccatcgacctgcccaccaacctgttcgacgccgagatcaagaacgacctgcagcacagcctgatccagaaccagatcccctacaacgagaccgacaccaacaaccagctgttcaagctgtggtggaccaaggtgaagaacaacggcttcatgaagttctacaacgccaagagggagtactgcatctacgacgagtacgtgaacttcgagatcaagccccagggcaagttcgccgactactacaagagcgccctgaagaccgccttcgagaagctggacaagcagagggagaccgagaggatcgccaacaaggccctgcccaaggtgcagatcaagcaggtggagaaggtgttcaagcagaccatcggcaacaccgagaaggagatcaggatcctgcaggaacaggacgccctgatgctgctgatgttcgagaagctgctgaacaatcccaaccccaatatcctggagaacatcagcatggagaacatcctgaacgagagcatcgacgtgaagatcgagatcaacggcaagctgagcttcgagaacgagggcgagatcatcaagaagaacgagaacaagccccagatcagcaggatcatcgtggagaagaggaagcggaaggagttcagcgtgctgcagaagtacctgcacgacaagaggctgcccgagctgttcgagtacttcgacaagcaggagatccccgtgagcgagctgaagctggagctcgacacctacaaccaggtgaagaaccaggtgttcgacctggtgttcaggttcgagaagaccctgatcgagaaggactacgagggcatcaagagcttcatcgagaccaagaccggcgaggagcccaagaaccacatccagcacaagccctacctgttctggctgaagagcaagaacttcatcgacgagaacgagttcaggttcctgaacatggtgaggaacaccttcagccacaaccagttccctcagaagaagaccatggacctgttcatcacccagtgggagaacaacaagttcgccaacgccatcttcgagttctacaagggcaaggtggagaacatcctgaacatcctga

SEQ ID NO: 13 - DNA, 4209 bp, unidentified
  source 1..4209: mol_type = other DNA
atgaacaccaccgacaagaggaccaagcccaactacaaggacttcatcaacgacaaggactacttcagcgcctacctgaacatggccaggcacaacgcctacatcaccgtggcccacatcagccacctgcttggcggaaagccctctggagatgacgccaagatcatggagatgaaggccatgcaggtgctgcagggcaccgacaacatcgagaagcagaagtgcatcaggcagctgaacaagcacttcaagttcctgcccgccgtggtgtactacgagaagctgtgggagaagaagaaggccgagaacaggttcgacatcctggacagcgagctggacaccgaggagagcttcgacctgcaggacagcaagcagcagcttagcgagggcaacatctactacagcgtgctgagcaagctgttcgagcccctgaacgacctgaggaacttctacacccactactaccaccccgtggtggtggtccccaactacgtgttcggcttcatgaacaagatcttcgacgccagcgtgaggatctgcaagcagaggttcggctacaacgagaaggacatcaagcacctgaggaggtacgacggcagcgagaccgacagcaccggaaaacggatgcccaaggagaaccctaggttcttcttcaagatcaacgagcccaacggcaccatcaccgagaagggcctggccttctacatctgcctgttcctggagaagaagtacgccagcaacttcctgaagaagctgaccggcttcaaggacgccaggaccgccgacaagcagagcacctttgaggtgtacaccgctctgaggatgcacctgcccaagcagaggatcaggagcgaggagaccaagctgggcatcgctctggacatgctgaacgagctgcagaagtgccccgacgagctgtacgagctgctgagcgacgagaaccaggacaagttcagggtggaggtgaccatgaggagcgacgccgacgactacgaggaaaacggcctgttcaagaggttcgacaacaggttcccctacttcgccctgaagtacttcgacttcagagccggcttccccatcaggttccacgtggacatgggcaagtactacttcaagttctacgagaagaagctggtgaacggcagcaccgagatcaggaagctggacaaggacctgagggccttcggaaggatcgccgagctggacgagtacaggaagaacgagtgggccgagctgatcaaggccaaccccgtgaacaccgagaactttgacttcgacaccgccaccagcgacaagtaccagccctacatccaggacacctaccctcactaccacatcgaggacaaccagatcggcctgaagttcaccgaggtggacatcgtgcccgagatcaacgccgagaagaccaggaaccagaagcccgacgcctacctgagcacctacgagttagccggcatgttcttctacgactggctcaacaagaacaaagagcagagcgccagcgctgtgctgctgaaggagtactacgacaaggtgaggaagctgttcgaggacatcggcaacgacaccatcaagcccatcaacttccagttcaccgccaacgctaacgacgagatctggcagaacgagctgaagcaggccaagatccaggccaacgagatcatcagcaagagctacaacctggacatccacaacctgcccgagatcatccagaggcacctgatcggcctgagcatcatcaaggacgacgccttcaagatctacgccgtggacaggatcaacaagatgctgggcgagaccgagagcaggctgaagaagctggacaagggcatcaggatcgccaacgacaagaagatcaagttcggcagcaagaggttcaaggagatcaagagcggcgtgctggccgacttcctggccaaggacctgatcaggtttcaacccaccgagcagaacggcaaggacaagatcaccggcctgaacttccagatcctgcaggcccacctggccaccttcaacgagaacaagcacctgctgcccagcatcttcaaggagtgcaagctgaccgacagcgtgatccagcaccccttcctgttcaagctgaaccccagcaagcacctggaccacatcagcttctgcaaggcctacctggtggagaggaagttctacctgcagaagtgcctgaaggaggccaagttcaacagctactacttcctgcagcagaagaggaagaacctgaacgagaggaagcagagcaacttcatcaagaacgtgaccaagaagtacctgaacgagcaccccatcaatttccctaggggcctgttctgcgaggccatcaggagcatgatcaagaaggacagcttcagccacttcaagaacctgaaccccaaggccagcgagaccagcatcaggaacttcctggagctgacccagaacaggaccaacaccgtgttcctgatccagaagtacttcgagctgctgaggggcgacgagagccaggagttctaccagtacgagaggagctacaagttcatcaaccagctgtacgacaggagggacaggaaccagatgaccaaggagctgccccagctgttctaccccgtgaaggacgtggtggagaatggcaggctgatcaccgaaggcctggtgagcatcgtggacaagctgaagaaggacatcaagaagctgcctcccatccctcagaccatcaagagcctgaggttcggcgagaagcctcccatgtacaaggagagcatgatggcccagtacaaccagttcaagaagaacgaggccaagctgaggctgtacaaggtgcaggacatgctgatcctgctgatcgccgagcacctgctggagctcgagaacattaacatccccagcggcctgttcctgctgaagaacatcctgcctcccgacctggtgaaccccgtggacgacaagaagaacatcctgaactaccccgtgaggtaccccatcaacctgcagttcaagaacctgcccgtggccaccatctaccagaacggcctgaagatcaagaacgtgggcgacttcgtgagattcaccagggacaggaggatcgagggcctgctggactggtacaggatcgactacttcaagcccaaggacgccaacggcaacatcgtggtggacaagaagggcaagcacctgctgtacaagggcaccgacaagttcgtgtacgagatcaaccggctgttcatcgagaacgagttcagcgtgtacgagaagctgaggatcgtggtgctgcagaacgtgctgaccttcgagaaggtgatgcacgacctgtacaagcccgagctgatcgccgagctggctgctgagaacgtgaggctgaagaccaagttcgacgccgaggaggccgagaagaaggccaacgccgagtctaagggagagatctacatcgtgaagcagtacagcgagatcaagtacttcgacttcaaggtggtgaccaacgtgttctacaacaagtaccaccagttcacccacgagagggacgccgtggtgcacctgaggaacaagttcgcccacaacgagttccccgagaagagcgtgctgacccagctggacgtgttccagaagatcgtggacgactaccccaacagcatcgagtacgccaacgagaagcaggccaggatcgacaacacccctgacatgcccgacgacgagaagaggatcgagaggctgaggatcgagcagctgaggagcatcaccgacaagatcgcccagcagagcaggatcctgttcgagaagtacatcgccgagatcaagagggaggagatcagcgccgaggctgagaccctgttcaacaccctgatcaagaacctgaacagcaatagcctggccaagatcagcaccgccatccagaccacctaccccgccgaaaacacacccctgaccatgtacagcagcgccttcgccgaagacagcaaggccgtgatcagcttcaggtactacagcgacagccaccccgagactgagaccaccgacgtgagccagaacatcaacagcatcatcagcaacgccaacagcctgggcctgtactacttcaacgagagcctgaggttcttcctgaacaacgcccagcccgagttcgaaatcgagaccatcaacagcgtgaagtaccccgacctcggcgacctgttcaacacccagatcatcggcaagtacagccagaagatcggcaagaacaacgag

SEQ ID NO: 14 - DNA, 3203 bp, unidentified
  source 1..3203: mol_type = other DNA
atggagaacaagaccgagagcctgagcaagaccatccagggcaaccccgcctacttcggagtgtacctgaacatggccaggcacaacatcctgctggtggacaaccacctggacaagaagttcaaccagaagaacagcatcaccgacgacgagaagatcagcgacagcttcctgaccaggaccaagagcgacaaccccaaccacctgtacagcgagctgatcaggtacatcccctgctgcagcatctacgaccccgagttcatggtgaccaacaaggagaagaaggaggacatggccatcatcgccagcatcgagaagggcaaggacttcaccaccatgcccgtgcacctgaaggccgtgttcaaggacatcaaccagctgaggaacagctacacccactacggccacaccgacaacaactgggagaggaaggccaagatcagcaccgagaccaaggagttcctggagagggtgtacagcaaggccatcaactacagccagaagaggttcaagaacgtgatccccgacgaggagttcaccaagctgaccaacctgcccatcttcctgcagaacgagcccagcaccctgacccaggacggattgatcttcctgaccagcctgttcctggagagggagttcatgttctacttcatcaaccagtgccacggcctgaagaacgccaccagcctgagcttcaagagcaagcgggagctgttcggcgttttctgcctcaggctgccccacgagaagatcatcagcgacgaccccaagaacgccctgttcctggacgtgctgaacgagatcaacaaggtgcccaaggagatcttcaaccacctgctgcccgagcagcagaaggagttcaggcccgacttctctgacgagaggaacgagaagatcgccgagaacagcatcagggaggacgaggaggacctggacacctacatccaggagctgcagaaccagtacaggagaggccagaggttctactacctggccaccaggctgatcgacgagctgaagatgctgcccgacttcaggttccagatcaggatcggcaagtacctgaagaagagcggccagaagaagttcggcaacgacatggtgaagagggagatcatcgacgacatcttcggattcggcagactggccgagttcatggacgagcagaagatcaccaccgccatcaacatcgacaaggtggaggaccagaggttcgagagcttcgcccctagctacgacctgaaggccaacaaggtgcagatcaagctgttcgccggcagcaacaccgccctggacgtggagaagatcaacaaggacggcaagaccgtgggctacacctacagcaacaaggtgttcagcatctccatccacgagctggtgaagatcctcatcctggagtacttcgagcccaaggccgccaaccagatcatcaaggacttcatcaacaagaacaggttcatcagcgacatcaaggagatcgagaagctgaaggccgagctggccagcatggacaacaagtacagaatctacgaggacaagaacaccagccccgagagactgagccagtacaaggagatgatggccgacaggaccagcctgctggacgccgctctgatcaagtttggcttggacagccagagcatccctagggccctggtggactacctgatcagcgtgaagcccagcaacaggagcttcgccatggtgaggaagatcaaggaggtgaagaacgaggccaggcagaaggtgagcgactacgacgagtacatcaggcccaagatcggcgagatggccaccgagatcgccaaggacatcatcgacatgatcatcagcaaggagaagaaggagaggtgcaccagcttctactacgacaagatgcaggaggccctggctctgtacgccagcgacgaaaagagggagctgttcgctcagatcgtgaaggacctgaacctgctggacgagaagcagggccaccccttcctgaagtacgtgagcttcaagagcttcaccaagaccggcgagttctacagggcctacttctacgccaaggccggcaagaagggcgaaaggggccaagacggctcttggatgtacaggaccttctacaccttcgacaggaagaccaagaagaccaccatccaggtgcccaacgagggcctgccctacatcttcaccaggcttcagaagccccacggcatcgctgacctgcagagctgggtgaacaacttcaacaagaccgccatcgacctgcccaccaacatcttcgacaagaagatcgaggaggccctgaagagcgagctgctgaagatcggcaaggtgagcgacggcaacgagaagtggagcgagctgttcaagaagtggtaccagagccagggcctgctgcagcccttctacaacctggagaggacctaccacgtgtatgactacgacttcaaggccggcagcgactacgacgacgcctacaaaaacaagatcgagcagctggccctgaagatcagccaggacaagaagaaggaggccaagggcaagttcgacatgcagtacaccaagcagaagatcaagcagctgctgcacaaggagatcacccacaacgagaggggcatcagggagatcgtggagcaggacatcgtgctggccatcaacctggaggtgccctaccagatcagggacctgcacaagatcaaggagcacctgaacgagaccatcctgctgagcgagaaggtggaggacaagaagatcgaggccaccaggaagagaaaggactacggcctgctgaacaagatcaggcacgacaagaggctgaagagcctgttcacctacatcgtggccgagaccgtggagtacgagaccgtgaagagcctgctgaaggagtacaacgacgtgaggatcaagatcttcgaccacgtgttcgccctggagaacctgatcctgagcaagtacaagaacgaggtggtgcaggagcagaagagcacctacggccccaacgacaccaacatcaagcacgacccctacctgaacgtgctgctgaccaagggcatcatcaccgacacagagaaggagatcctgaagaccatcagggacaagttcagccacaacgaggtgcccgtgctggacgaggtggacaaggactgcatcttcgagagcatgtacaggatccacgccaccatcatcaacaagatcaccgacagcctgaccacccacag

SEQ ID NO: 15 - DNA, 2904 bp, unidentified
  source 1..2904: mol_type = other DNA
atgttcctgtacaagaacgaggccaacgagctgatcagcaagatcaagggcttcaagaggagcgacgacaacaccttcaggagcaagaggaacctgttcagcttctacagcaagaagttcagcagccaggacatcgacagcgaggagggcaacctgatcaagttcagggacatcgtgcagtacctgaacctgtaccccaagcactggaacagcgagctggagttcgacgccaagatccctcagatgaccaagcccctgaaggacaagatcgtggaaatggagatcgagaggtgcttccccaagaaggacgagaaggacgagctgttctaccccaagtacgacaggctgttcaacgacagctacgagaagttcaagatctacgccaagtaccagatcttcggcaagaagttcctgggcaaggtgatcgagaacgagtacatcaagcaggacttcagcgacttcgagctggacatcttcagcttcgagatcaacaagaccaagaagtacaaggacagcttcaggaaggagaagagcttcgagaagaggaagaaggacctggagtacaagagcttccacaagaagagcgaggaggacttcctgaagaactaccagaagaacctgaaggacatccagaggatcatcgaggaggagaaagagaaccttaacctggacacccagaagctgcagaagaggatcgcccagaacatgctgcacgtgcagtacggcaggaaccaggacaggttcatggacttcgccatcaggttcctggccgagaagaagtacttcggcaacgaggccgagttcaagatctaccagttccacaccaccgacgagcagaacaactgcctggccacccagggcaaagtgctgaccaagaaggagttcgacaacctgaagtaccaccagggcaagctggtggtgtacaagagcttcgaggagcacctgaagaagtaccccgactgggacacccctttcgtgatcgagaacaacagcttccacgtgaagatcaacttctgctgcgccagcaagatcatctgcatccagaggaacgccctgatctacctgctggagcacgccctgtacggcaacaacgcccagaccatcgagaacgctggcaaggagctgctgatcaagtacttcgtggagaacgagaccgccttcgacaagaagtacaacatcctgaagaccaacaccgagatcagcaaggacgagaagaccgagctgaagaagttcttccccaagaggctgctgcacaactactacaaggacgagaccagcgtgaagaagaccaagacaagcagcctgcagaagatcctggacgacgccaacgaggccgaaaccaggtaccagaagctgctggtgaaggtcaagagggaggagaccgagtacaaggccaagtaccccgaggacgacaccgttgccctggttgccaacttcgagaagaggaacaagggcaagcagttcaagctgaggttcatgaggaaggcctggcagctgatgtacttcaaggacgcctacctgaagcagatccaggccgacaacaagcaccacaagagctacaacatcagcagggacgagttcaacgacttcagcaagtggctgtacgccttcgaggagatccccgtgtacaaggagtacctgagcgacatgttcgcccagaagaccttcttcgtgaacaaggagttcaaggacctgttcgacaggagcaccaccttcgagaacctgtacagcaagaccaaggagaggtacaccaactggctgaagaccaacgacaccgccctgcagaagaccttcgagctgaagaactacgagaccctgctgagcaggaccaccctgttcattaacatcaacaggttcatcgacttcctggtgagggagggcaagctgaccaagaacagcgagaacatgttcgagtacaagagcctggagaactggggctacctgatcgagaagtactacttcaaggagaagctggagaagaccgagtacaagacctgcggcaagctgttcaacaagctgaggaccgtgaagctggaggactgcctgctgtacgagatggccatcgactacctgcagaccgacaagaccatcgccgaccacgccaagaagcacatcagggtgctgcagaccaaggacgtgatcatcgaggtgcccgacatcaacaccaacaacggcggcctgttcaagctggagatccccttcaacaagctgatggccttcgaggagctgttcaagcagaaggaagaggaggagaacgagcccaagaacaggaagaccagcttcctgagcaacatccagatctacctgaagaagctgaaggagatgagcgagaagaccaaggacaagagggagatcgagaagggcatcagcgacaccgtgacctacttcaacgccaacaagggcctgaagttcgagcacctgaacaagatctacagccacctgatcagcaccagcgccaagttcaccaaggtggagctcgagctggagaagtacttcatcgtgaagaacaaggtggagatccccaaccacgagaacaggatcaccttcgacgacatcgacgccaaaaaggagaaggtgctgagcaagtacttcgacaagaccatcaggaagaaggccttccacttcggcgtgcccatcatcgagaacaagcccttcacctacaaggagaagctggacgagattgagatcaagttcatccagaacgaggtgaagcccctgaacaagaagagcttcgacgagtacgagcccgagatgaagagcgtgctgatcgccctgctggagacccttcacgacgccttctacgagaagaactactacgagaacggcaagaagagggagaaggacggcaagaagaaggtggccgacgccaagaacaagtacttcaacgaggtgatcatcaagaag

SEQ ID NO: 16 - DNA, 1629 bp, unidentified
  source 1..1629: mol_type = other DNA
atggccgacttcgtggctcgggacatgatccggctgcagaagaacatcggcaaggacggaggcaagcccaacagcaccgagttccagatcctgcaggccaagctggctttcttcggcaagaacaaggacaccctgcacgacaccttcaagctgttcaagctgatcgacagcgagaaccagcaccccttcctgaacaagatcgacatcaacagcaccaacggcatcctggacttctacaaggagtacctgagccagcggaagaagtacctcgagcagtgcatcagcgagaagaagtacgacgagtaccacttcctgaagctgggcgacaagcagaagcagagcggccagaagcacatcgaggagctggccaccaagctgaagaacgaggtcgtgatgaacctgcccaggggactgttcctgaagcctatcctggaggccctgaagagcagcgagaagaccaacaagctggccctggagctggagaataccggacgcgtgaacaccgcctacatcatcgaccagtacttcaccaagatcatgaacgacaagagccaggagctgtacggctacagcaagagctacgagttcctgaacaagatcttcgacaaccggaaggaggacaagatgcggaacaccctgcccagcaagtacttcaccaccgaggagctgaccaagatgaccatcaacaacgagatcgagaacaagctgcacgagagcatcaccaagcagatcaagaagaagcggatcaacaacgagatcgagatcgagcggatcaaggaggtgtacaagaagggctacaagtacttcaccaacaacgagaagcagatccggctggtgaagaccaccgacaagatcctgttcatgatggccgacgaggtgttccggaaggagttcgtgaccgacaacggcctgatcaagagccggaagaacaacagcagccagtaccagaccagcgtgtccatcgacatcgggtacaagctggccgagatcagacccgatagcgacaagggcatcctgagcctgaggaccaaggtgtccctgatcatgccctacacctacgagaccaagaaggacaagatcgtgggcctggacaacgccaagagcatcagaagcgagaacaagatcaagaccatcgtgaacgagaccatcaagatcaagaactacggcaacttccggggcttcctgaaggacagacggatcagcagcctgatgccctacatcaccgacaacgaggtgcagttcgaggccgtgaagaaggagctggaggagtttggcaaggccaggatcgagatcttcaagaagatctacgagttcgagaagatcgtgatcaaggagaaggagctgaacctgaacgccatcccctacatcaaccacggcgacatcctgaagagcctgatcgacgagaaggacgagcggttcatcatcatcaagcagctgcgggacgcctttagccacagcaactaccccgactacctgctgttcgagaacgacatcaacggcgagggcttcaacgagctgaagaactacaccagcaagcggaaggacatcctgaacaacagcatcgcctaccagttcaagaacctgaccatcaagtactacgacgagctgatcaagctggccaccggcaag

SEQ ID NO: 17 - DNA, 2535 bp, unidentified
  source 1..2535: mol_type = other DNA
atgaacgaggagtggaagaagcggttcctgcccaagctggaggagcagcagaaggagaacctgcagaagaactctagcccagccgaggaggagatcgagaactacgacaagttcatggagctgctgaccaagcaggtccgacacgcagatcggttcagcatcttcgccatgcggttcatcgacgagatgcagctgttcgacacttggcgcttccacatcaacctgggcaagatcctgctggccagctaccagaagcacctgaacggagaggacgtggacaggctgatcgtggaagacgtgaaggccttcggcagactgaacgactacccctacgagagcaagatcatcaacaagatcaaccggaccgacgaccccatggtgaagttcgagcagttcgtgccccactaccacgccgagaacaacaagatcggcctctgcaggaaccggaagaccctgggcccagtgatgatcgagaaccaggacgcccagagcaagaacaagcggaacatcaagcagccccaccccgaagtgtttctgagcctgcacgagctgcccaagatcatcctgctggagtacctgaagaagggcgagaccgagaggctgatcaacgagttcgtggccctgaacaacagcagcctcatgaaccgggagttcatcgacgagatcaagaccaaggtgccccaggattggaacggcttccagaagaagaccagcagcgagaagagcagcggctacagagaggaggcactgaagtacctgcagggccggaagaagatcctgaacgacgtgctggccgcctacaacctgaacgaccggcagatccccaccaagatcctcaactactggctgaacatccaggacgtgcctctggacagggtgctgagcgagcggatcaagaagatgcggaaggattgcaagcagcggctgaaggccctgagaaagtacaggagggagggcaagggcagaatccccaaagtgggagagatggcctccttcctggccaaggacatcgtggacatggtcatcggcgaggagaagaagaagaagatcaccagcttctactacgacaagatgcaggagtgcctggctctgtacgccgatccagagaagaaggccctgttcatcgacatcgtcaacaacgagctgcacctgaacgagaccgacggacatcccttcctgaagaacgtgcccaggagcgaagtgtcctacaccaccgacatctacgagcgctacctggaggagaagggctacaaggagatcgaggtcaccaacgagaagaccggcaagaggaccaagcgggacgtgtcttggatggagaagaccttctacaagaaggagcgggaccccaagaccggcaagctgaagaccaacgtgggcatcttcagcgacggcaacgccattcctctgaccatcaggcggagcagcgagaagatcagcgagtctctggacgattggctggcccacgtgaagaacggcttcaagcccatcgacggcagcagacctatcgacctgcccaccaacctgttcgacgagaccatcaacgccctgctgaagaacgacctgaagaagcacaacgtgctgagcagcgaggacgccaagtggaacgagctgttcaagctctggtggagcgaagtgcggaaggacagcacacaggactattacaccgcccccagggagtacatgatctacgacgagaaggtctgcttcagcaacaccggcaagggcaagtacagcgagtactacggaagcgccgtggaagccgcctattctaagaagaacgccgagcaggaggagaagcggaagaagaaccccaggctgcccaagatcgagcgctgccagatcgagaaggtgttcagcaagaccatcggcaagaccgagaaggagatccggatcgtggaggagaaggacaggagcctgctgctgatgatcgagcagctgctgagcgaccagggagccaagaccgagaacctgaagctgaaggagtacgtgcggctgctggatcaggaagtgaccatcaggatccccttcccagtgcctcagcagaaggagggagaggcttgtcccgagaaggacatcgtgaccaagcggaagcggaaggactacggagccctgcagcggttcatcagcgataggaggctgccaggcctgtacgagtacttcccaggagacgagatccccatggacgatctggaggtggagctggacgcctacaacaaggccaagcagaacgtgctggacagggccttccagctggagaagaacatcatcgaccgggacatggtgcgcgtgtcagagctgttcggcaagatcagcaacatccagcacaagccctacgtcgactggctgaaggagaagagcctgatcgacgaggaaatcgacagcttcctgaacgccgtgcggaacaagttcagccacaacgagtacccccccaagggcatcatggagaacgtgatcaagaagtgggacgagaaggcctacgcctctcagatcgaggaggcctacagccaggagatcaacaagatcctgatgcagctg

SEQ ID NO: 18 - DNA, 2550 bp, unidentified
  source 1..2550: mol_type = other DNA
atgtgcaggctgaagaacggcaggctgagggccgccatcttcgccaagatcgtgatcttctggtaccagaacttcaggatgaggctgcacgtgaacaagagcaagatgaagcagggcagcgtgttcaacgccgccaccgacaagatccccttcgccatcttcttcaacagggcccaggagaggctgaacggctggtacggcagcctggactctatcaacgccgacatcaccgtgagcaagcaggacttcaccagctggttcaagcagttcaagagcgaggagggcaacatgatgcccgagaagaggcagctggtgaaggacaaggtgatcgccaggctgaaggacgtgttcaggttcgccgactacctgttcaggtggaacatgagcaacagcatcctgaagctgatcgacaagctgaacgacctgaggaacttcttcagccacggctaccacaggcccgtggagtggagcgagtacgagattgacaccctgaacaagctgtacttcagcctgagcgagtacaggcccaagctgaacaggcagaacctggagaactgcctgctgttcgacgagaacaagaccctgagctaccagggcgccatcttcttcgtgagcctgttcctgaccaaggaggacgtgaaccagctgttcgacctgatctacttctgcttcagggccgagaagaacctgcccgccgactctctgcctcacaggttcctgaacttcaaccctaggagggagatctacaccttctggaacaggaggggcgacgccagcctgatgcctgacaatcggcagctgaagaagttctacgacatcgtgagcttcctgaggaagtgccccgaggagagcctgacccctgaaaccgagaagctggctgagaagtacggcgtgagggagagcgacaagttcatcaggcacgccatggactacctgagcgacttcaaggccctgcccaacctggagttcttcccctataagaacaagaaggagatcttcaggggcaacaccctgttcctgctgagggacgacaagcacggctgcctgaagggcatgatgggcgaagaggtgctgaccagggtgttggtgaggctgttcagcggcatccccggaaccagcatcgagaccgagattagggagttcatcaggacctactacgagaacagcctgctgaccatcgacagcttcacccaccccgtgcccaagagcgttgacaggaagagaaagatcgccgaaggcgacaacctgctgttcgaggtgctggacgagaggatcctgaggaggctggagttcatcagctacaggctgaaggacctgaagagggagagcaccagcttcagcgagagccagaaggccgacttcatcgttaggaggtggaacaggtggatcatgtacaacttcaagaaggccgacggcgtggacaagagcatcaagaacatccagttcatcaagctgagggcccagctgaccaacttcaggaagttcaagagggagatcatcaacgagctggccgccagcggctacgacaaggtgtaccccatcaaggagctgttggaggagagcgacctggagaccctgtacaagaagaccatcgagtacgacggcaagttctgcgacaagttcctggccaacgagaatgagaggaggaagaaggccgaggccatctgcaagtacgtgggcctgaggcccatcaagatcggagtgagcgagagcaacatgagcaagatgcccgtgcccatcgcccctaaggccatcagctgcgacaggttgaagttcgagaagaccctggtggacctgatcgacgagtactaccccatcaggaccggcctgaacaagacccacaaggacaacaagcccgccatcagcaaggagaggagagtgaacaagaagtactggaagctgaagcagagggacagcctgctggccctgatcgccagcgaatacctgaggaacggcatcaagaagaccgccgagatcggcaggatcagcctgtacaggttcgacgaggacatcgtggaactgaagctgaaactggactacaccctgcagttcgaggacaagaccgccgacaccatcaaggccaagaagctgagcttcaccttcgacgagttcgccaagagcaggaacaggatgatcctgggcggcctgaaggacatcgccttcagcaacaagttccccgacaacgagatcgactacagccacatcgagcccgagctggagacctacctgtacagccagatcgagttcatgaggaagatcctggagctggaagagaggctgctgaagcagaagcccgagctgaaggtgctgagcaagaagtacgtgcccttcggcgacatcgagaagaacctggacaacctgagcaggcacttcgacaagttcaaggccgcctaccccaccgacatgacccacatcgacaaccttaggaggatcttcaggaacagcgccctgcacatgagcgtgcccaagatcgacgacaaggtgcttgtgggctacttccagcagggcatcgacttcatcaactactacatcgagcagcagttcggctga

SEQ ID NO: 19 - DNA, 65 bp, unidentified
  source 1..65: mol_type = other DNA
gttgtagctgtctttatttgaaaggcacagacaaccccatggttttcttctgcattacggggccg

SEQ ID NO: 20 - RNA, 37 nt, unidentified
  source 1..37: mol_type = other RNA
ggtgcagtcgcccttcacttgggcgtggtgttgcgac

SEQ ID NO: 21 - RNA, 36 nt, unidentified
  source 1..36: mol_type = other RNA
gttgtaactgccttgattttgtaaggtataaacaac

SEQ ID NO: 22 - RNA, 36 nt, unidentified
  source 1..36: mol_type = other RNA
gttgtagaagcccttgtttttaagggtaggcacaac

SEQ ID NO: 23 - RNA, 37 nt, unidentified
  source 1..37: mol_type = other RNA
gtctgaagagttcacagtttggtggatgcttgcagac

SEQ ID NO: 24 - RNA, 36 nt, unidentified
  source 1..36: mol_type = other RNA
gttgtttataccttacaaaatcaaggcagttacaac

SEQ ID NO: 25 - RNA, 36 nt, unidentified
  source 1..36: mol_type = other RNA
gctgtaactacctttcaaaatcaaggcttccacagc

SEQ ID NO: 26 - RNA, 35 nt, unidentified
  source 1..35: mol_type = other RNA
gttgtagctgtctttatttgaaaggcacagacaac

SEQ ID NO: 27 - RNA, 37 nt, unidentified
  source 1..37: mol_type = other RNA
gccgttcccaccttacaaacgcaaggcttccacagct

SEQ ID NO: 28 - DNA, 715 bp, unidentified
  source 1..715: mol_type = other DNA
ggtgagcaagggcgaggagctgttcaccggggtggtgcccatcctggtcgagctggacggcgacgtaaacggccacaagttcagcgtgcgcggcgagggcgagggcgatgccaccaacggcaagctgaccctgaagttcatctgcaccaccggcaagctgcccgtgccctggcccaccctcgtgaccaccctgacctacggcgtgcagtgcttcagccgctaccccgaccacatgaagcgccacgacttcttcaagtccgccatgcccgaaggctacgtccaggagcgcaccatcagcttcaaggacgacggcacctacaagacccgcgccgaggtgaagttcgagggcgacaccctggtgaaccgcatcgagctgaagggcatcgacttcaaggaggacggcaacatcctggggcacaagctggagtacaacttcaacagccacaacgtctatatcaccgccgacaagcagaagaacggcatcaaggccaacttcaagatccgccacaacgtggaggacggcagcgtgcagctcgccgaccactaccagcagaacacccccatcggcgacggccccgtgctgctgcccgacaaccactacctgagcacccagtccaagctgagcaaagaccccaacgagaagcgcgatcacatggtcctgctggagttcgtgaccgccgccgggatcactcacggcatggacgagctgtacaag

SEQ ID NO: 29 - DNA, 12019 bp, unidentified
  source 1..12019: mol_type = other DNA
tggaagggctaattcactcccaaagaagacaagatatccttgatctgtggatctaccacacacaaggctacttccctgattagcagaactacacaccagggccaggggtcagatatccactgacctttggatggtgctacaagctagtaccagttgagccagataaggtagaagaggccaataaaggagagaacaccagcttgttacaccctgtgagcctgcatgggatggatgacccggagagagaagtgttagagtggaggtttgacagccgcctagcatttcatcacgtggcccgagagctgcatccggagtacttcaagaactgctgatatcgagcttgctacaagggactttccgctggggactttccagggaggcgtggcctgggcgggactggggagtggcgagccctcagatcctgcatataagcagctgctttttgcctgtactgggtctctctggttagaccagatctgagcctgggagctctctggctaactagggaacccactgcttaagcctcaataaagcttgccttgagtgcttcaagtagtgtgtgcccgtctgttgtgtgactctggtaactagagatccctcagacccttttagtcagtgtggaaaatctctagcagtggcgcccgaacagggacttgaaagcgaaagggaaaccagaggagctctctcgacgcaggactcggcttgctgaagcgcgcacggcaagaggcgaggggcggcgactggtgagtacgccaaaaattttgactagcggaggctagaaggagagagatgggtgcgagagcgtcagtattaagcgggggagaattagatcgcgatgggaaaaaattcggttaaggccagggggaaagaaaaaatataaattaaaacatatagtatgggcaagcagggagctagaacgattcgcagttaatcctggcctgttagaaacatcagaaggctgtagacaaatactgggacagctacaaccatcccttcagacaggatcagaagaacttagatcattatataatacagtagcaaccctctattgtgtgcatcaaaggatagagataaaagacaccaaggaagctttagacaagatagaggaagagcaaaacaaaagtaagaccaccgcacagcaagcggccggccgctgatcttcagacctggaggaggagatatgagggacaattggagaagtgaattatataaatataaagtagtaaaaattgaaccattaggagtagcacccaccaaggcaaagagaagagtggtgcagagagaaaaaagagcagtgggaataggagctttgttccttgggttcttgggagcagcaggaagcactatgggcgcagcgtcaatgacgctgacggtacaggccagacaattattgtctggtatagtgcagcagcagaacaatttgctgagggctattgaggcgcaacagcatctgttgcaactcacagtctggggcatcaagcagctccaggcaagaatcctggctgtggaaagatacctaaaggatcaacagctcctggggatttggggttgctctggaaaactcatttgcaccactgctgtgccttggaatgctagttggagtaataaatctctggaacagatttggaatcacacgacctggatggagtgggacagagaaattaacaattacacaagcttaatacactccttaattgaagaatcgcaaaaccagcaagaaaagaatgaacaagaattattggaattagataaatgggcaagtttgtggaattggtttaacataacaaattggctgtggtatataaaattattcataatgatagtaggaggcttggtaggtttaagaatagtttttgctgtactttctatagtgaatagagttaggcagggatattcaccattatcgtttcagacccacctcccaaccccgaggggacccgacaggcccgaaggaatagaagaagaaggtggagagagagacagagacagatccattcgattagtgaacggatctcgacggtatcgccgaattcacaaatggcagtattcatccacaattttaaaagaaaaggggggattggggggtacagtgcaggggaaagaatagtagacataatagcaacagacatacaaactaaagaattacaaaaacaaattacaaaaattcaaaattttcgggtttattacagggacagcagagatccagtttggactagtcgtgaggctccggtgcccgtcagtgggcagagcgcacatcgcccacagtccccgagaagttggggggaggggtcggcaattgaaccggtgcctagagaaggtggcgcggggtaaactgggaaagtgatgtcgtgtactggctccgcctttttcccgagggtgggggagaaccgtatataagtgcagtagtcgccgtgaacgttctttttcgcaacgggtttgccgccagaacacaggtaagtgccgtgtgtggttcccgcgggcctggcctctttacgggttatggcccttgcgtgccttgaattacttccacgcccctggctgcagtacgtgattcttgatcccgagcttcgggttggaagtgggtgggagagttcgaggccttgcgcttaaggagccccttcgcctcgtgcttgagttgaggcctggcctgggcgctggggccgccgcgtgcgaatctggtggcaccttcgcgcctgtctcgctgctttcgataagtctctagccatttaaaatttttgatgacctgctgcgacgctttttttctggcaagatagtcttgtaaatgcgggccaagatctgcacactggtatttcggtttttggggccgcgggcggcgacggggcccgtgcgtcccagcgcacatgttcggcgaggcggggcctgcgagcgcggccaccgagaatcggacgggggtagtctcaagctggccggcctgctctggtgcctggcctcgcgccgccgtgtatcgccccgccctgggcggcaaggctggcccggtcggcaccagttgcgtgagcggaaagatggccgcttcccggccctgctgcagggagctcaaaatggaggacgcggcgctcgggagagcgggcgggtgagtcacccacacaaaggaaaagggcctttccgtcctcagccgtcgcttcatgtgactccacggagtaccgggcgccgtccaggcacctcgattagttctcgagcttttggagtacgtcgtctttaggttggggggaggggttttatgcgatggagtttccccacactgagtgggtggagactgaagttaggccagcttggcacttgatgtaattctccttggaatttgccctttttgagtttggatcttggttcattctcaagcctcagacagtggttcaaagtttttttcttccatttcaggtgtcgtgaagcggccgcatgaagcgacctgccgccacaaagaaggctggacaggctaagaagaagaaagctagcatcgagaagaagaagagcttcgccaagggcatgggcgtgaagagcaccctggtgtccggctctaaggtgtacatgaccacatttgccgagggctccgacgcacggctggagaagatcgtggagggcgatagcatcagatccgtgaacgagggagaggccttcagcgccgagatggccgacaagaatgccggctataagatcggcaacgccaagttttcccacccaaagggctatgccgtggtggccaacaatccactgtacaccggaccagtgcagcaggacatgctgggcctgaaggagacactggagaagagatacttcggcgagagcgccgacggcaatgataacatctgcatccaggtcatccacaatatcctggatatcgagaagatcctggccgagtatatcaccaacgccgcctacgccgtgaacaatatctccggcctggacaaggatatcatcggcttcggcaagttttctaccgtgtacacatatgacgagttcaaggaccccgagcaccacagggccgcctttaacaataacgacaagctgatcaatgccatcaaggcccagtacgacgagttcgataattttctggataacccccggctgggctattttggccaggccttcttttctaaggagggcagaaactatatcatcaattacggcaacgagtgttacgacatcctggccctgctgagcggactgaggcactgggtggtgcacaataacgaggaggagtctaggatcagccgcacctggctgtataatctggacaagaatctggataacgagtacatctccacactgaactacctgtatgatcggatcaccaatgagctgacaaacagcttctccaagaattctgccgccaatgtgaactacatcgcagagaccctgggcatcaacccagcagagttcgcagagcagtacttccggttcagcatcatgaaggagcagaagaatctgggctttaacatcacaaagctgcgggaagtgatgctggacagaaaggatatgtccgagatccggaagaaccacaaggtgttcgattctatcagaaccaaggtgtatacaatgatggactttgtgatctaccggtactatatcgaggaggatgccaaggtggccgccgccaataagagcctgcccgacaacgagaagtctctgagcgagaaggatatcttcgtgatcaatctgagaggctcctttaacgacgatcagaaggacgccctgtactatgatgaggccaatcggatctggagaaagctggagaatatcatgcacaacatcaaggagttcaggggcaacaagacccgcgagtacaagaagaaggacgcaccaaggctgcctcgcatcctgcctgcaggaagggacgtgagcgccttcagcaagctgatgtatgccctgacaatgtttctggacggcaaggagatcaatgatctgctgaccacactgatcaataagttcgacaacatccagtcctttctgaaagtgatgcctctgatcggcgtgaacgccaagttcgtggaggagtacgccttctttaaggacagcgccaagatcgccgatgagctgaggctgatcaagtcctttgccaggatgggagagccaatcgcagacgcaaggagagccatgtacatcgatgccatcagaatcctgggcaccaatctgtcttatgatgagctgaaggccctggccgacaccttcagcctggacgagaatggcaacaagctgaagaagggcaagcacggcatgcgcaatttcatcatcaataacgtgatcagcaacaagaggtttcactatctgatcagatacggcgaccctgcacacctgcacgagatcgccaagaacgaggccgtggtgaagttcgtgctgggcaggatcgccgatatccagaagaagcagggccagaatggcaagaaccagatcgaccgctactatgagacctgcatcggcaaggataagggcaagtccgtgtctgagaaggtggacgccctgaccaagatcatcacaggcatgaattatgaccagttcgataagaagcggagcgtgatcgaggacaccggaagggagaacgcagagagagagaagtttaagaagatcatcagcctgtatctgacagtgatctaccacatcctgaagaatatcgtgaatatcaacgccagatacgtgatcggcttccactgcgtggagcgcgatgcccagctgtataaggagaagggctacgacatcaacctgaagaagctggaggagaagggctttagctccgtgaccaagctgtgcgcaggaatcgacgagacagcacccgacaagcggaaggatgtggagaaggagatggccgagagagccaaggagagcatcgactccctggagtctgccaatcctaagctgtacgccaactatatcaagtactccgatgagaagaaggccgaggagttcacccggcagatcaatagagagaaggccaagaccgccctgaacgcctacctgcggaatacaaagtggaacgtgatcatcagggaggacctgctgcgcatcgataataagacctgtacactgttcaggaacaaggccgtgcacctggaggtggcccgctatgtgcacgcctacatcaatgacatcgccgaggtgaactcctactttcagctgtaccactatatcatgcagcggatcatcatgaacgagagatatgagaagtctagcggcaaggtgtctgagtacttcgacgccgtgaatgatgagaagaagtataacgatagactgctgaagctgctgtgcgtgcctttcggctactgtatcccaaggtttaagaatctgagcatcgaggccctgttcgacaggaacgaggcagccaagtttgataaggagaagaagaaggtgagcggcaactccagtctagaggtgagcaagggcgaggagctgttcaccggggtggtgcccatcctggtcgagctggacggcgacgtaaacggccacaagttcagcgtgcgcggcgagggcgagggcgatgccaccaacggcaagctgaccctgaagttcatctgcaccaccggcaagctgcccgtgccctggcccaccctcgtgaccaccctgacctacggcgtgcagtgcttcagccgctaccccgaccacatgaagcgccacgacttcttcaagtccgccatgcccgaaggctacgtccaggagcgcaccatcagcttcaaggacgacggcacctacaagacccgcgccgaggtgaagttcgagggcgacaccctggtgaaccgcatcgagctgaagggcatcgacttcaaggaggacggcaacatcctggggcacaagctggagtacaacttcaacagccacaacgtctatatcaccgccgacaagcagaagaacggcatcaaggccaacttcaagatccgccacaacgtggaggacggcagcgtgcagctcgccgaccactaccagcagaacacccccatcggcgacggccccgtgctgctgcccgacaaccactacctgagcacccagtccaagctgagcaaagaccccaacgagaagcgcgatcacatggtcctgctggagttcgtgaccgccgccgggatcactcacggcatggacgagctgtacaagtaccccaagaaaaagcgcaaggtacgcgtgcagctaagcgactacaaagaccatgacggtgattataaagatcatgacatcgattacaaggatgacgatgacaagtaaggatccctcccccccccctaacgttactggccgaagccgcttggaataaggccggtgtgcgtttgtctatatgttattttccaccatattgccgtcttttggcaatgtgagggcccggaaacctggccctgtcttcttgacgagcattcctaggggtctttcccctctcgccaaaggaatgcaaggtctgttgaatgtcgtgaaggaagcagttcctctggaagcttcttgaagacaaacaacgtctgtagcgaccctttgcaggcagcggaaccccccacctggcgacaggtgcctctgcggccaaaagccacgtgtataagatacacctgcaaaggcggcacaaccccagtgccacgttgtgagttggatagttgtggaaagagtcaaatggctctcctcaagcgtattcaacaaggggctgaaggatgcccagaaggtaccccattgtatgggatctgatctggggcctcggtgcacatgctttacatgtgtttagtcgaggttaaaaaaacgtctaggccccccgaaccacggggacgtggttttcctttgaaaaacacgatgataaggatccaccggagcttaccatgaccgagtacaagcccacggtgcgcctcgccacccgcgacgacgtccccagggccgtacgcaccctcgccgccgcgttcgccgactaccccgccacgcgccacaccgtcgatccggaccgccacatcgagcgggtcaccgagctgcaagaactcttcctcacgcgcgtcgggctcgacatcggcaaggtgtgggtcgcggacgacggcgccgcggtggcggtctggaccacgccggagagcgtcgaagcgggggcggtgttcgccgagatcggcccgcgcatggccgagttgagcggttcccggctggccgcgcagcaacagatggaaggcctcctggcgccgcaccggcccaaggagcccgcgtggttcctggccaccgtcggcgtctcgcccgaccaccagggcaagggtctgggcagcgccgtcgtgctccccggagtggaggcggccgagcgcgccggggtgcccgccttcctggagacctccgcgccccgcaacctccccttctacgagcggctcggcttcaccgtcaccgccgacgtcgaggtgcccgaaggaccgcgcacctggtgcatgacccgcaagcccggtgcctgacgcccatcgatagatcctaatcaacctctggattacaaaatttgtgaaagattgactggtattcttaactatgttgctccttttacgctatgtggatacgctgctttaatgcctttgtatcatgctattgcttcccgtatggctttcattttctcctccttgtataaatcctggttgctgtctctttatgaggagttgtggcccgttgtcaggcaacgtggcgtggtgtgcactgtgtttgctgacgcaacccccactggttggggcattgccaccacctgtcagctcctttccgggactttcgctttccccctccctattgccacggcggaactcatcgccgcctgccttgcccgctgctggacaggggctcggctgttgggcactgacaattccgtggtgttgtcggggaaatcatcgtcctttccttggctgctcgcctgtgttgccacctggattctgcgcgggacgtccttctgctacgtcccttcggccctcaatccagcggaccttccttcccgcggcctgctgccggctctgcggcctcttccgcgtcttcgccttcgccctcagacgagtcggatctccctttgggccgcctccccgcctgagatcctttaagaccaatgacttacaaggcagctgtagatcttagccactttttaaaagaaaaggggggactggaagggctaattcactcccaacgaagacaagatctgctttttgcttgtactgggtctctctggttagaccagatctgagcctgggagctctctggctaactagggaacccactgcttaagcctcaataaagcttgccttgagtgcttcaagtagtgtgtgcccgtctgttgtgtgactctggtaactagagatccctcagacccttttagtcagtgtggaaaatctctagcagtagtagttcatgtcatcttattattcagtatttataacttgcaaagaaatgaatatcagagagtgagaggcccgggttaattaaggaaagggctagatcattcttgaagacgaaagggcctcgtgatacgcctatttttataggttaatgtcatgataataatggtttcttagacgtcaggtggcacttttcggggaaatgtgcgcggaacccctatttgtttatttttctaaatacattcaaatatgtatccgctcatgagacaataaccctgataaatgcttcaataatattgaaaaaggaagagtatgagtattcaacatttccgtgtcgcccttattcccttttttgcggcattttgccttcctgtttttgctcacccagaaacgctggtgaaagtaaaagatgctgaagatcagttgggtgcacgagtgggttacatcgaactggatctcaacagcggtaagatccttgagagttttcgccccgaagaacgttttccaatgatgagcacttttaaagttctgctatgtggcgcggtattatcccgtgttgacgccgggcaagagcaactcggtcgccgcatacactattctcagaatgacttggttgagtactcaccagtcacagaaaagcatcttacggatggcatgacagtaagagaattatgcagtgctgccataaccatgagtgataacactgcggccaacttacttctgacaacgatcggaggaccgaaggagctaaccgcttttttgcacaacatgggggatcatgtaactcgccttgatcgttgggaaccggagctgaatgaagccataccaaacgacgagcgtgacaccacgatgcctgtagcaatggcaacaacgttgcgcaaactattaactggcgaactacttactctagcttcccggcaacaattaatagactggatggaggcggataaagttgcaggaccacttctgcgctcggcccttccggctggctggtttattgctgataaatctggagccggtgagcgtgggtctcgcggtatcattgcagcactggggccagatggtaagccctcccgtatcgtagttatctacacgacggggagtcaggcaactatggatgaacgaaatagacagatcgctgagataggtgcctcactgattaagcattggtaactgtcagaccaagtttactcatatatactttagattgatttaaaacttcatttttaatttaaaaggatctaggtgaagatcctttttgataatctcatgaccaaaatcccttaacgtgagttttcgttccactgagcgtcagaccccgtagaaaagatcaaaggatcttcttgagatcctttttttctgcgcgtaatctgctgcttgcaaacaaaaaaaccaccgctaccagcggtggtttgtttgccggatcaagagctaccaactctttttccgaaggtaactggcttcagcagagcgcagataccaaatactgttcttctagtgtagccgtagttaggccaccacttcaagaactctgtagcaccgcctacatacctcgctctgctaatcctgttaccagtggctgctgccagtggcgataagtcgtgtcttaccgggttggactcaagacgatagttaccggataaggcgcagcggtcgggctgaacggggggttcgtgcacacagcccagcttggagcgaacgacctacaccgaactgagatacctacagcgtgagctatgagaaagcgccacgcttcccgaagggagaaaggcggacaggtatccggtaagcggcagggtcggaacaggagagcgcacgagggagcttccagggggaaacgcctggtatctttatagtcctgtcgggtttcgccacctctgacttgagcgtcgatttttgtgatgctcgtcaggggggcggagcctatggaaaaacgccagcaacgcggcctttttacggttcctggccttttgctggccttttgctcacatgttctttcctgcgttatcccctgattctgtggataaccgtattaccgcctttgagtgagctgataccgctcgccgcagccgaacgaccgagcgcagcgagtcagtgagcgaggaagcggaagagcgcccaatacgcaaaccgcctctccccgcgcgttggccgattcattaatgcagcaagctcatggctgactaattttttttatttatgcagaggccgaggccgcctcggcctctgagctattccagaagtagtgaggaggcttttttggaggcctaggcttttgcaaaaagctccccgtggcacgacaggtttcccgactggaaagcgggcagtgagcgcaacgcaattaatgtgagttagctcactcattaggcaccccaggctttacactttatgcttccggctcgtatgttgtgtggaattgtgagcggataacaatttcacacaggaaacagctatgacatgattacgaatttcacaaataaagcatttttttcactgcattctagttgtggtttgtccaaactcatcaatgtatcttatcatgtctggatcaactggataactcaagctaaccaaaatcatcccaaacttcccaccccataccctattaccactgccaattacctgtggtttcatttactctaaacctgtgattcctctgaattattttcattttaaagaaattgtatttgttaaatatgtactacaaacttagtagt

SEQ ID NO: 30 - DNA, 6080 bp, unidentified
  source 1..6080: mol_type = other DNA
gacggatcgggagatctcccgatcccctatggtgcactctcagtacaatctgctctgatgccgcatagttaagccagtatctgctccctgcttgtgtgttggaggtcgctgagtagtgcgcgagcaaaatttaagctacaacaaggcaaggcttgaccgacaattgcatgaagaatctgcttagggttaggcgttttgcgctgcttcgcgatgtacgggccagatatacgcgttgacattgattattgactagttattaatagtaatcaattacggggtcattagttcatagcccatatatggagttccgcgttacataacttacggtaaatggcccgcctggctgaccgcccaacgacccccgcccattgacgtcaataatgacgtatgttcccatagtaacgccaatagggactttccattgacgtcaatgggtggagtatttacggtaaactgcccacttggcagtacatcaagtgtatcatatgccaagtacgccccctattgacgtcaatgacggtaaatggcccgcctggcattatgcccagtacatgaccttatgggactttcctacttggcagtacatctacgtattagtcatcgctattaccatggtgatgcggttttggcagtacatcaatgggcgtggatagcggtttgactcacggggatttccaagtctccaccccattgacgtcaatgggagtttgttttggcaccaaaatcaacgggactttccaaaatgtcgtaacaactccgccccattgacgcaaatgggcggtaggcgtgtacggtgggaggtctatataagcagagctctctggctaactagagaacccactgcttactggcttatcgaaattaatacgactcactatagggagacccaagcttggtaccatggtgagcaagggcgaggaggataacatggccatcatcaaggagttcatgcgcttcaaggtgcacatggagggctccgtgaacggccacgagttcgagatcgagggcgagggcgagggccgcccctacgagggcacccagaccgccaagctgaaggtgaccaagggtggccccctgcccttcgcctgggacatcctgtcccctcagttcatgtacggctccaaggcctacgtgaagcaccccgccgacatccccgactacttgaagctgtccttccccgagggcttcaagtgggagcgcgtgatgaacttcgaggacggcggcgtggtgaccgtgacccaggactcctccctgcaggacggcgagttcatctacaaggtgaagctgcgcggcaccaacttcccctccgacggccccgtaatgcagaagaaaaccatgggctgggaggcctcctccgagcggatgtaccccgaggacggcgccctgaagggcgagatcaagcagaggctgaagctgaaggacggcggccactacgacgctgaggtcaagaccacctacaaggccaagaagcccgtgcagctgcccggcgcctacaacgtcaacatcaagttggacatcacctcccacaacgaggactacaccatcgtggaacagtacgaacgcgccgagggccgccactccaccggcggcatggacgagctgtacaagctcgagcatgcatctagagggccctattctatagtgtcacctaaatgctagagctcgctgatcagcctcgactgtgccttctagttgccagccatctgttgtttgcccctcccccgtgccttccttgaccctggaaggtgccactcccactgtcctttcctaataaaatgaggaaattgcatcgcattgtctgagtaggtgtcattctattctggggggtggggtggggcaggacagcaagggggaggattgggaagacaatagcaggcatgctggggatgcggtgggctctatggcttctgaggcggaaagaaccagctggggctctagggggtatccccacgcgccctgtagcggcgcattaagcgcggcgggtgtggtggttacgcgcagcgtgaccgctacacttgccagcgccctagcgcccgctcctttcgctttcttcccttcctttctcgccacgttcgccggctttccccgtcaagctctaaatcgggggctccctttagggttccgatttagtgctttacggcacctcgaccccaaaaaacttgattagggtgatggttcacgtagtgggccatcgccctgatagacggtttttcgccctttgacgttggagtccacgttctttaatagtggactcttgttccaaactggaacaacactcaaccctatctcggtctattcttttgatttataagggattttgccgatttcggcctattggttaaaaaatgagctgatttaacaaaaatttaacgcgaattaattctgtggaatgtgtgtcagttagggtgtggaaagtccccaggctccccagcaggcagaagtatgcaaagcatgcatctcaattagtcagcaaccaggtgtggaaagtccccaggctccccagcaggcagaagtatgcaaagcatgcatctcaattagtcagcaaccatagtcccgcccctaactccgcccatcccgcccctaactccgcccagttccgcccattctccgccccatggctgactaattttttttatttatgcagaggccgaggccgcctctgcctctgagctattccagaagtagtgaggaggcttttttggaggcctaggcttttgcaaaaagctcccgggagcttgtatatccattttcggatctgatcaagagacaggatgaggatcgtttcgcatgattgaacaagatggattgcacgcaggttctccggccgcttgggtggagaggctattcggctatgactgggcacaacagacaatcggctgctctgatgccgccgtgttccggctgtcagcgcaggggcgcccggttctttttgtcaagaccgacctgtccggtgccctgaatgaactgcaggacgaggcagcgcggctatcgtggctggccacgacgggcgttccttgcgcagctgtgctcgacgttgtcactgaagcgggaagggactggctgctattgggcgaagtgccggggcaggatctcctgtcatctcaccttgctcctgccgagaaagtatccatcatggctgatgcaatgcggcggctgcatacgcttgatccggctacctgcccattcgaccaccaagcgaaacatcgcatcgagcgagcacgtactcggatggaagccggtcttgtcgatcaggatgatctggacgaagagcatcaggggctcgcgccagccgaactgttcgccaggctcaaggcgcgcatgcccgacggcgaggatctcgtcgtgacccatggcgatgcctgcttgccgaatatcatggtggaaaatggccgcttttctggattcatcgactgtggccggctgggtgtggcggaccgctatcaggacatagcgttggctacccgtgatattgctgaagagcttggcggcgaatgggctgaccgcttcctcgtgctttacggtatcgccgctcccgattcgcagcgcatcgccttctatcgccttcttgacgagttcttctgagcgggactctggggttcgaaatgaccgaccaagcgacgcccaacctgccatcacgagatttcgattccaccgccgccttctatgaaaggttgggcttcggaatcgttttccgggacgccggctggatgatcctccagcgcggggatctcatgctggagttcttcgcccaccccaacttgtttattgcagcttataatggttacaaataaagcaatagcatcacaaatttcacaaataaagcatttttttcactgcattctagttgtggtttgtccaaactcatcaatgtatcttatcatgtctgtataccgtcgacctctagctagagcttggcgtaatcatggtcatagctgtttcctgtgtgaaattgttatccgctcacaattccacacaacatacgagccggaagcataaagtgtaaagcctggggtgcctaatgagtgagctaactcacattaattgcgttgcgctcactgcccgctttccagtcgggaaacctgtcgtgccagctgcattaatgaatcggccaacgcgcggggagaggcggtttgcgtattgggcgctcttccgcttcctcgctcactgactcgctgcgctcggtcgttcggctgcggcgagcggtatcagctcactcaaaggcggtaatacggttatccacagaatcaggggataacgcaggaaagaacatgtgagcaaaaggccagcaaaaggccaggaaccgtaaaaaggccgcgttgctggcgtttttccataggctccgcccccctgacgagcatcacaaaaatcgacgctcaagtcagaggtggcgaaacccgacaggactataaagataccaggcgtttccccctggaagctccctcgtgcgctctcctgttccgaccctgccgcttaccggatacctgtccgcctttctcccttcgggaagcgtggcgctttctcatagctcacgctgtaggtatctcagttcggtgtaggtcgttcgctccaagctgggctgtgtgcacgaaccccccgttcagcccgaccgctgcgccttatccggtaactatcgtcttgagtccaacccggtaagacacgacttatcgccactggcagcagccactggtaacaggattagcagagcgaggtatgtaggcggtgctacagagttcttgaagtggtggcctaactacggctacactagaagaacagtatttggtatctgcgctctgctgaagccagttaccttcggaaaaagagttggtagctcttgatccggcaaacaaaccaccgctggtagcggtttttttgtttgcaagcagcagattacgcgcagaaaaaaaggatctcaagaagatcctttgatcttttctacggggtctgacgctcagtggaacgaaaactcacgttaagggattttggtcatgagattatcaaaaaggatcttcacctagatccttttaaattaaaaatgaagttttaaatcaatctaaagtatatatgagtaaacttggtctgacagttaccaatgcttaatcagtgaggcacctatctcagcgatctgtctatttcgttcatccatagttgcctgactccccgtcgtgtagataactacgatacgggagggcttaccatctggccccagtgctgcaatgataccgcgagacccacgctcaccggctccagatttatcagcaataaaccagccagccggaagggccgagcgcagaagtggtcctgcaactttatccgcctccatccagtctattaattgttgccgggaagctagagtaagtagttcgccagttaatagtttgcgcaacgttgttgccattgctacaggcatcgtggtgtcacgctcgtcgtttggtatggcttcattcagctccggttcccaacgatcaaggcgagttacatgatcccccatgttgtgcaaaaaagcggttagctccttcggtcctccgatcgttgtcagaagtaagttggccgcagtgttatcactcatggttatggcagcactgcataattctcttactgtcatgccatccgtaagatgcttttctgtgactggtgagtactcaaccaagtcattctgagaatagtgtatgcggcgaccgagttgctcttgcccggcgtcaatacgggataataccgcgccacatagcagaactttaaaagtgctcatcattggaaaacgttcttcggggcgaaaactctcaaggatcttaccgctgttgagatccagttcgatgtaacccactcgtgcacccaactgatcttcagcatcttttactttcaccagcgtttctgggtgagcaaaaacaggaaggcaaaatgccgcaaaaaagggaataagggcgacacggaaatgttgaatactcatactcttcctttttcaatattattgaagcatttatcagggttattgtctcatgagcggatacatatttgaatgtatttagaaaaataaacaaataggggttccgcgcacatttccccgaaaagtgccacctgacgtc

SEQ ID NO: 31 - DNA, 708 bp, unidentified
  source 1..708: mol_type = other DNA
atggtgagcaagggcgaggaggataacatggccatcatcaaggagttcatgcgcttcaaggtgcacatggagggctccgtgaacggccacgagttcgagatcgagggcgagggcgagggccgcccctacgagggcacccagaccgccaagctgaaggtgaccaagggtggccccctgcccttcgcctgggacatcctgtcccctcagttcatgtacggctccaaggcctacgtgaagcaccccgccgacatccccgactacttgaagctgtccttccccgagggcttcaagtgggagcgcgtgatgaacttcgaggacggcggcgtggtgaccgtgacccaggactcctccctgcaggacggcgagttcatctacaaggtgaagctgcgcggcaccaacttcccctccgacggccccgtaatgcagaagaaaaccatgggctgggaggcctcctccgagcggatgtaccccgaggacggcgccctgaagggcgagatcaagcagaggctgaagctgaaggacggcggccactacgacgctgaggtcaagaccacctacaaggccaagaagcccgtgcagctgcccggcgcctacaacgtcaacatcaagttggacatcacctcccacaacgaggactacaccatcgtggaacagtacgaacgcgccgagggccgccactccaccggcggcatggacgagctgtacaag

SEQ ID NO: 32 - DNA, 2914 bp, unidentified
  source 1..2914: mol_type = other DNA
tcgcgcgtttcggtgatgacggtgaaaacctctgacacatgcagctcccggagacggtcacagcttgtctgtaagcggatgccgggagcagacaagcccgtcagggcgcgtcagcgggtgttggcgggtgtcggggctggcttaactatgcggcatcagagcagattgtactgagagtgcaccagatgcggtgtgaaataccgcacagatgcgtaaggagaaaataccgcatcaggcgccattcgccattcaggctgcgcaactgttgggaagggcgatcggtgcgggcctcttcgctattacgccagctggcgaaagggggatgtgctgcaaggcgattaagttgggtaacgccagggttttcccagtcacgacgttgtaaaacgacggccagtgagggcctatttcccatgattccttcatatttgcatatacgatacaaggctgttagagagataattggaattaatttgactgtaaacacaaagatattagtacaaaatacgtgacgtagaaagtaataatttcttgggtagtttgcagttttaaaattatgttttaaaatggactatcatatgcttaccgtaacttgaaagtatttcgatttcttggctttatatatcttgtggaaaggacgaaacaccgagtcttcgatattcaagcgtcggaagactcgttttggcgtaatcatggtcatagctgtttcctgtgtgaaattgttatccgctcacaattccacacaacatacgagccggaagcataaagtgtaaagcctggggtgcctaatgagtgagctaactcacattaattgcgttgcgctcactgcccgctttccagtcgggaaacctgtcgtgccagctgcattaatgaatcggccaacgcgcggggagaggcggtttgcgtattgggcgctcttccgcttcctcgctcactgactcgctgcgctcggtcgttcggctgcggcgagcggtatcagctcactcaaaggcggtaatacggttatccacagaatcaggggataacgcaggaaagaacatgtgagcaaaaggccagcaaaaggccaggaaccgtaaaaaggccgcgttgctggcgtttttccataggctccgcccccctgacgagcatcacaaaaatcgacgctcaagtcagaggtggcgaaacccgacaggactataaagataccaggcgtttccccctggaagctccctcgtgcgctctcctgttccgaccctgccgcttaccggatacctgtccgcctttctcccttcgggaagcgtggcgctttctcatagctcacgctgtaggtatctcagttcggtgtaggtcgttcgctccaagctgggctgtgtgcacgaaccccccgttcagcccgaccgctgcgccttatccggtaactatcgtcttgagtccaacccggtaagacacgacttatcgccactggcagcagccactggtaacaggattagcagagcgaggtatgtaggcggtgctacagagttcttgaagtggtggcctaactacggctacactagaagaacagtatttggtatctgcgctctgctgaagccagttaccttcggaaaaagagttggtagctcttgatccggcaaacaaaccaccgctggtagcggtggtttttttgtttgcaagcagcagattacgcgcagaaaaaaaggatctcaagaagatcctttgatcttttctacggggtctgacgctcagtggaacgaaaactcacgttaagggattttggtcatgagattatcaaaaaggatcttcacctagatccttttaaattaaaaatgaagttttaaatcaatctaaagtatatatgagtaaacttggtctgacagttaccaatgcttaatcagtgaggcacctatctcagcgatctgtctatttcgttcatccatagttgcctgactccccgtcgtgtagataactacgatacgggagggcttaccatctggccccagtgctgcaatgataccgcgactcccacgctcaccggctccagatttatcagcaataaaccagccagccggaagggccgagcgcagaagtggtcctgcaactttatccgcctccatccagtctattaattgttgccgggaagctagagtaagtagttcgccagttaatagtttgcgcaacgttgttgccattgctacaggcatcgtggtgtcacgctcgtcgtttggtatggcttcattcagctccggttcccaacgatcaaggcgagttacatgatcccccatgttgtgcaaaaaagcggttagctccttcggtcctccgatcgttgtcagaagtaagttggccgcagtgttatcactcatggttatggcagcactgcataattctcttactgtcatgccatccgtaagatgcttttctgtgactggtgagtactcaaccaagtcattctgagaatagtgtatgcggcgaccgagttgctcttgcccggcgtcaatacgggataataccgcgccacatagcagaactttaaaagtgctcatcattggaaaacgttcttcggggcgaaaactctcaaggatcttaccgctgttgagatccagttcgatgtaacccactcgtgcacccaactgatcttcagcatcttttactttcaccagcgtttctgggtgagcaaaaacaggaaggcaaaatgccgcaaaaaagggaataagggcgacacggaaatgttgaatactcatactcttcctttttcaatattattgaagcatttatcagggttattgtctcatgagcggatacatatttgaatgtatttagaaaaataaacaaataggggttccgcgcacatttccccgaaaagtgccacctgacgtctaagaaaccattattatcatgacattaacctataaaaataggcgtatcacgaggccctttcgtc

SEQ ID NO: 33 - DNA, 30 bp, unidentified
  source 1..30: mol_type = other DNA
gcagcttcaccttgtagatgaactcgccgt

SEQ ID NO: 34 - DNA, 30 bp, unidentified
  source 1..30: mol_type = other DNA
gttcatcacgcgctcccacttgaagccctc

SEQ ID NO: 35 - DNA, 30 bp, unidentified
  source 1..30: mol_type = other DNA
tgcttcacgtaggccttggagccgtacatg

SEQ ID NO: 36 - DNA, 30 bp, unidentified
  source 1..30: mol_type = other DNA
tcagcttggcggtctgggtgccctcgtagg

SEQ ID NO: 37 - DNA, 30 bp, unidentified
  source 1..30: mol_type = other DNA
ttgatgatggccatgttatcctcctcgccc

SEQ ID NO: 38 - DNA, 30 bp, unidentified
  source 1..30: mol_type = other DNA
cccatggttttcttctgcattacggggccg

SEQ ID NO: 39 - DNA, 30 bp, unidentified
  source 1..30: mol_type = other DNA
caggatgtcccaggcgaagggcagggggcc

SEQ ID NO: 40 - DNA, 30 bp, unidentified
  source 1..30: mol_type = other DNA
tgtagatgaactcgccgtcctgcagggagg

SEQ ID NO: 41 - DNA, 30 bp, unidentified
  source 1..30: mol_type = other DNA
ttcagcctctgcttgatctcgcccttcagg

SEQ ID NO: 42 - DNA, 30 bp, unidentified
  source 1..30: mol_type = other DNA
cctcagcgtcgtagtggccgccgtccttca

SEQ ID NO: 43 - DNA, 30 bp, unidentified
  source 1..30: mol_type = other DNA
cgtctggccttcctgtagccagctttcatc

SEQ ID NO: 44 - DNA, 30 bp, unidentified
  source 1..30: mol_type = other DNA
ttaggcagccctcatcagtgccggctccct

SEQ ID NO: 45 - DNA, 30 bp, unidentified
  source 1..30: mol_type = other DNA
ggccaggatctcaattaggcagccctcatc

SEQ ID NO: 46 - DNA, 30 bp, unidentified
  source 1..30: mol_type = other DNA
atggcccttcgcagctcttgcacgtcatac

SEQ ID NO: 47 - DNA, 30 bp, unidentified
  source 1..30: mol_type = other DNA
cctcctgaccagaagctgcctgaaggctca

SEQ ID NO: 48 - DNA, 30 bp, unidentified
  source 1..30: mol_type = other DNA
ctggtatacctcctgaccagaagctgcctg

SEQ ID NO: 49 - DNA, 30 bp, unidentified
  source 1..30: mol_type = other DNA
caaatgctggtaacactgtggtccacaagg

SEQ ID NO: 50 - DNA, 30 bp, unidentified
  source 1..30: mol_type = other DNA
gagagcagcagcaaactcctttgctccctc

SEQ ID NO: 51 - DNA, 30 bp, unidentified
  source 1..30: mol_type = other DNA
tttgctccctccaaatgctggtaacactgt

SEQ ID NO: 52 - DNA, 30 bp, unidentified
  source 1..30: mol_type = other DNA
ggcccgtagtgcttcagtttgaagttctca

SEQ ID NO: 53 - DNA, 30 bp, unidentified
  source 1..30: mol_type = other DNA
gcttcagtttgaagttctcatcggggaagc

SEQ ID NO: 54 - DNA, 30 bp, unidentified
  source 1..30: mol_type = other DNA
cctactaggaccataggtacatcttcagag

SEQ ID NO: 55 - DNA, 30 bp, unidentified
  source 1..30: mol_type = other DNA
gtgtctactgttctagaaggcaaatcacat

SEQ ID NO: 56 - DNA, 2898 bp, unidentified
  source 1..2898: mol_type = other DNA
atcgagaagaagaagagcttcgccaagggcatgggcgtgaagagcaccctggtgtccggctctaaggtgtacatgaccacatttgccgagggctccgacgcacggctggagaagatcgtggagggcgatagcatcagatccgtgaacgagggagaggccttcagcgccgagatggccgacaagaatgccggctataagatcggcaacgccaagttttcccacccaaagggctatgccgtggtggccaacaatccactgtacaccggaccagtgcagcaggacatgctgggcctgaaggagacactggagaagagatacttcggcgagagcgccgacggcaatgataacatctgcatccaggtcatccacaatatcctggatatcgagaagatcctggccgagtatatcaccaacgccgcctacgccgtgaacaatatctccggcctggacaaggatatcatcggcttcggcaagttttctaccgtgtacacatatgacgagttcaaggaccccgagcaccacagggccgcctttaacaataacgacaagctgatcaatgccatcaaggcccagtacgacgagttcgataattttctggataacccccggctgggctattttggccaggccttcttttctaaggagggcagaaactatatcatcaattacggcaacgagtgttacgacatcctggccctgctgagcggactgaggcactgggtggtgcacaataacgaggaggagtctaggatcagccgcacctggctgtataatctggacaagaatctggataacgagtacatctccacactgaactacctgtatgatcggatcaccaatgagctgacaaacagcttctccaagaattctgccgccaatgtgaactacatcgcagagaccctgggcatcaacccagcagagttcgcagagcagtacttccggttcagcatcatgaaggagcagaagaatctgggctttaacatcacaaagctgcgggaagtgatgctggacagaaaggatatgtccgagatccggaagaaccacaaggtgttcgattctatcagaaccaaggtgtatacaatgatggactttgtgatctaccggtactatatcgaggaggatgccaaggtggccgccgccaataagagcctgcccgacaacgagaagtctctgagcgagaaggatatcttcgtgatcaatctgagaggctcctttaacgacgatcagaaggacgccctgtactatgatgaggccaatcggatctggagaaagctggagaatatcatgcacaacatcaaggagttcaggggcaacaagacccgcgagtacaagaagaaggacgcaccaaggctgcctcgcatcctgcctgcaggaagggacgtgagcgccttcagcaagctgatgtatgccctgacaatgtttctggacggcaaggagatcaatgatctgctgaccacactgatcaataagttcgacaacatccagtcctttctgaaagtgatgcctctgatcggcgtgaacgccaagttcgtggaggagtacgccttctttaaggacagcgccaagatcgccgatgagctgaggctgatcaagtcctttgccaggatgggagagccaatcgcagacgcaaggagagccatgtacatcgatgccatcagaatcctgggcaccaatctgtcttatgatgagctgaaggccctggccgacaccttcagcctggacgagaatggcaacaagctgaagaagggcaagcacggcatgcgcaatttcatcatcaataacgtgatcagcaacaagaggtttcactatctgatcagatacggcgaccctgcacacctgcacgagatcgccaagaacgaggccgtggtgaagttcgtgctgggcaggatcgccgatatccagaagaagcagggccagaatggcaagaaccagatcgaccgctactatgagacctgcatcggcaaggataagggcaagtccgtgtctgagaaggtggacgccctgaccaagatcatcacaggcatgaattatgaccagttcgataagaagcggagcgtgatcgaggacaccggaagggagaacgcagagagagagaagtttaagaagatcatcagcctgtatctgacagtgatctaccacatcctgaagaatatcgtgaatatcaacgccagatacgtgatcggcttccactgcgtggagcgcgatgcccagctgtataaggagaagggctacgacatcaacctgaagaagctggaggagaagggctttagctccgtgaccaagctgtgcgcaggaatcgacgagacagcacccgacaagcggaaggatgtggagaaggagatggccgagagagccaaggagagcatcgactccctggagtctgccaatcctaagctgtacgccaactatatcaagtactccgatgagaagaaggccgaggagttcacccggcagatcaatagagagaaggccaagaccgccctgaacgcctacctgcggaatacaaagtggaacgtgatcatcagggaggacctgctgcgcatcgataataagacctgtacactgttcaggaacaaggccgtgcacctggaggtggcccgctatgtgcacgcctacatcaatgacatcgccgaggtgaactcctactttcagctgtaccactatatcatgcagcggatcatcatgaacgagagatatgagaagtctagcggcaaggtgtctgagtacttcgacgccgtgaatgatgagaagaagtataacgatagactgctgaagctgctgtgcgtgcctttcggctactgtatcccaaggtttaagaatctgagcatcgaggccctgttcgacaggaacgaggcagccaagtttgataaggagaagaagaaggtgagcggcaactcc

SEQ ID NO: 57 - DNA, 36 bp, unidentified
  source 1..36: mol_type = other DNA
caagtaaacccctaccaactggtcggggtttgaaac

SEQ ID NO: 58 - DNA, 66 bp, unidentified
  source 1..66: mol_type = other DNA
caagtaaacccctaccaactggtcggggtttgaaacgcagcttcaccttgtagatgaactcgccgt

SEQ ID NO: 59 - DNA, 66 bp, unidentified
  source 1..66: mol_type = other DNA
gttgtttataccttacaaaatcaaggcagttacaacgcagcttcaccttgtagatgaactcgccgt

SEQ ID NO: 60 - DNA, 67 bp, unidentified
  source 1..67: mol_type = other DNA
gccgttcccaccttacaaacgcaaggcttccacagctgcagcttcaccttgtagatgaactcgccgt

SEQ ID NO: 61 - DNA, 66 bp, unidentified
  source 1..66: mol_type = other DNA
caagtaaacccctaccaactggtcggggtttgaaaccccatggttttcttctgcattacggggccg

SEQ ID NO: 62 - DNA, 66 bp, unidentified
  source 1..66: mol_type = other DNA
gttgtaactgccttgattttgtaaggtataaacaaccccatggttttcttctgcattacggggccg

SEQ ID NO: 63 - DNA, 66 bp, unidentified
  source 1..66: mol_type = other DNA
gctgtaactacctttcaaaatcaaggcttccacagccccatggttttcttctgcattacggggccg